European Patent Application EP 4 230 654 A1, published August 23, 2023. Title: COMBINATION THERAPIES TARGETING PD-1, TIM-3, AND LAG-3. Applicant: SYMPHOGEN A/S. The sequence listing filed with the application follows.

SEQUENCE LISTING (397 sequences)

SEQ ID NO: 1 - DNA, 360 bp, synthetic construct
  misc_feature 1..360: note = source = /note="Description of Artificial Sequence: Synthetic polynucleotide"
  source 1..360: mol_type = other DNA
caggtgcagctacagcagtcgggcccaggactggtgaagccttcacagaccctgtccctcacctgcactgtctctggtggctccatcagcagtggtggttactactggagttggacccgtcagcacccagggatgggcctggagtggattggatacatctcttacagtgggagtatctattacactccgtccctcaagagtcgacttaccatatcagtggacacgtctaagaaccagttctccctgaagctgagctctgtgactgccgcggacacggccgtatattactgtgcgagtttggattcctggggatctaaccgtgactactggggccagggaaccctggtcaccgtctcgagt

SEQ ID NO: 2 - DNA, 321 bp, synthetic construct
  misc_feature 1..321: note = source = /note="Description of Artificial Sequence: Synthetic polynucleotide"
  source 1..321: mol_type = other DNA
gaaattgtgttgacgcagtctccagccaccctgtctttgtctccaggggaaagagccaccctctcctgcagggccagtcagagtgttagcagctacttagcctggtaccaacagaaacctggccaggctcccaggctcctcatctatgatgcatccaacagggccactggcatcccagccaggttcagtggcagtgggtctgggacagacttcactctcaccatcagcagcctagagcctgaagattttgcagtttattactgtcagcagcgtagcaactggccgctcactttcggcggagggaccaaggtggagattaag

SEQ ID NO: 3 - protein, 120 aa, synthetic construct
  REGION 1..120: note = source = /note="Description of Artificial Sequence: Synthetic polypeptide"
QVQLQQSGPGLVKPSQTLSLTCTVSGGSISSGGYYWSWTRQHPGMGLEWIGYISYSGSIYYTPSLKSRLTISVDTSKNQFSLKLSSVTAADTAVYYCASLDSWGSNRDYWGQGTLVTVSS

SEQ ID NO: 4 - protein, 107 aa, synthetic construct
  REGION 1..107: note = source = /note="Description of Artificial Sequence: Synthetic polypeptide"
EIVLTQSPATLSLSPGERATLSCRASQSVSSYLAWYQQKPGQAPRLLIYDASNRATGIPARFSGSGSGTDFTLTISSLEPEDFAVYYCQQRSNWPLTFGGGTKVEIK

SEQ ID NO: 5 - DNA, 360 bp, synthetic construct
  misc_feature 1..360: note = source = /note="Description of Artificial Sequence: Synthetic polynucleotide"
  source 1..360: mol_type = other DNA
caggtgcagctgcaggagagtggccccggactggtcaagccttcacagactctgagcctgacctgcacagtgtctggcggaagtatcagctccgggggttactattggagctggacccgacagcacccaggaatgggtctggaatggatcgggtacatttcatatagcggctccatctactatacaccctcactgaaaagcaggctgaccatttccgtggacacatctaagaaccagttcagcctgaaactgtctagtgtgacagccgctgatactgcagtctactattgtgcctccctggactcttggggcagtaatagagattactggggccagggaactctggtcaccgtctcgagt

SEQ ID NO: 6 - DNA, 321 bp, synthetic construct
  misc_feature 1..321: note = source = /note="Description of Artificial Sequence: Synthetic polynucleotide"
  source 1..321: mol_type = other DNA
gagatcgtgctgactcagtccccagccaccctgtcactgagcccaggagaacgagcaaccctgtcttgcagggcctcccagtctgtcagctcctacctggcttggtatcagcagaagcccgggcaggcacctcgactgctgatctacgacgccagtaacagagctaccggtattcccgcccgcttcagtggttcaggcagcggaacagactttaccctgacaatctctagtctggagcctgaagatttcgccgtgtactattgtcagcagaggtctaattggccactgacatttggcggagggactaaggtcgagatcaag

SEQ ID NO: 7 - protein, 120 aa, synthetic construct
  REGION 1..120: note = source = /note="Description of Artificial Sequence: Synthetic polypeptide"
QVQLQESGPGLVKPSQTLSLTCTVSGGSISSGGYYWSWTRQHPGMGLEWIGYISYSGSIYYTPSLKSRLTISVDTSKNQFSLKLSSVTAADTAVYYCASLDSWGSNRDYWGQGTLVTVSS

SEQ ID NO: 8 - protein, 10 aa, synthetic construct
  REGION 1..10: note = source = /note="Description of Artificial Sequence: Synthetic peptide"
GGSISSGGYY

SEQ ID NO: 9 - protein, 7 aa, synthetic construct
  REGION 1..7: note = source = /note="Description of Artificial Sequence: Synthetic peptide"
ISYSGSI

SEQ ID NO: 10 - protein, 14 aa, synthetic construct
  REGION 1..14: note = source = /note="Description of Artificial Sequence: Synthetic peptide"
CASLDSWGSNRDYW

SEQ ID NO: 11 - protein, 6 aa, synthetic construct
  REGION 1..6: note = source = /note="Description of Artificial Sequence: Synthetic peptide"
QSVSSY

SEQ ID NO: 12 - skipped

SEQ ID NO: 13 - protein, 11 aa, synthetic construct [sequence omitted]

SEQ ID NO: 14 - DNA, 345 bp, synthetic construct
  misc_feature 1..345: note = source = /note="Description of Artificial Sequence: Synthetic polynucleotide"
  source 1..345: mol_type = other DNA
caggtcaccttgaaggagtggggcgcaggactgttgaggccctcggagaccctgtccctcacctgcgctgtctatggtgggtccttcagtggttactactggagctggatccgccagcccccagggaaggggctggagtggataggggaaatcaatcatagtggaagcaccaactacaacccgtccctcaagagtcgagtcaccatatcagtagacgcgaccaagaaacaattctccctgaagctgacctctgtgaccgccgcggacacggctgtgtattactgtgcgagatattgggagctccctgactactggggccagggcaccctggtcaccgtctcgagt

SEQ ID NO: 15 - DNA, 321 bp, synthetic construct
  misc_feature 1..321: note = source = /note="Description of Artificial Sequence: Synthetic polynucleotide"
  source 1..321: mol_type = other DNA
gacatccagttgacccagtctccatcctccctgtctgcatctgtaggagacagagtcaccatcacttgccgggcaagtcagggcattagaaatgatttaggctggtatcagcagaaaccagggaaagcccctaagcgcctgatctatgctgcatccagtttgcaaagtggggtcccatcaaggttcagcggcagtggatctgggacagaattcactctcacaatcagcagcctgcagcctgaagattttgcaacttattactgtctacagcataatagttaccctccgacgttcggccaagggaccaaggtggaaatcaag

SEQ ID NO: 16 - protein, 115 aa, synthetic construct
  REGION 1..115: note = source = /note="Description of Artificial Sequence: Synthetic polypeptide"
QVTLKEWGAGLLRPSETLSLTCAVYGGSFSGYYWSWIRQPPGKGLEWIGEINHSGSTNYNPSLKSRVTISVDATKKQFSLKLTSVTAADTAVYYCARYWELPDYWGQGTLVTVSS

SEQ ID NO: 17 - protein, 107 aa, synthetic construct
  REGION 1..107: note = source = /note="Description of Artificial Sequence: Synthetic polypeptide"
DIQLTQSPSSLSASVGDRVTITCRASQGIRNDLGWYQQKPGKAPKRLIYAASSLQSGVPSRFSGSGSGTEFTLTISSLQPEDFATYYCLQHNSYPPTFGQGTKVEIK

SEQ ID NO: 18 - protein, 8 aa, synthetic construct
  REGION 1..8: note = source = /note="Description of Artificial Sequence: Synthetic peptide"
GGSFSGYY

SEQ ID NO: 19 - protein, 7 aa, synthetic construct
  REGION 1..7: note = source = /note="Description of Artificial Sequence: Synthetic peptide"
INHSGST

SEQ ID NO: 20 - protein, 11 aa, synthetic construct
  REGION 1..11: note = source = /note="Description of Artificial Sequence: Synthetic peptide"
CARYWELPDYW

SEQ ID NO: 21 - protein, 6 aa, synthetic construct
  REGION 1..6: note = source = /note="Description of Artificial Sequence: Synthetic peptide"
QGIRND

SEQ ID NO: 22 - skipped

SEQ ID NO: 23 - protein, 11 aa, synthetic construct [sequence omitted]

SEQ ID NO: 24 - DNA, 345 bp, synthetic construct
  misc_feature 1..345: note = source = /note="Description of Artificial Sequence: Synthetic polynucleotide"
  source 1..345: mol_type = other DNA
cagatgcagctggtgcagtggggcgcaggactgttgaagccttcggagaccctgtccctcacctgcgctgtctatggtgggtccttcagtggttactactggagctggatccgccagcccccagggaaggggctggagtggattggggaaatcaatcatagtggaagcaccaactacaacccgtccctcaagagtcgagtcaccatgtcagttgacacgtccaagcaccagttctccctgaagctgagctctgtgaccgccgcggacacggctgtgtattactgtgcgagatggtgggagcttcctgactactggggccagggaaccctggtcaccgtctcgagt

SEQ ID NO: 25 - DNA, 321 bp, synthetic construct
  misc_feature 1..321: note = source = /note="Description of Artificial Sequence: Synthetic polynucleotide"
  source 1..321: mol_type = other DNA
gaaattgtgttgacgcagtctccatcctccctgtctgcatctgtaggagacagagtcaccatcacttgccgggcaagtcagggcattagaaatgatttaggctggtatcagcagaaaccagggaaagcccctaagcgcctgatctatgctgcatccagtttgcaaagtggggtcccatcaaggttcagcggcagtggatctgggacagaattcactctcacaatcagcagcctgcagcctgaagattttgcaacttattactgtctacagcataatagttacccgtggacgttcggccaagggaccaaggtggaaatcaag

SEQ ID NO: 26 - protein, 115 aa, synthetic construct
  REGION 1..115: note = source = /note="Description of Artificial Sequence: Synthetic polypeptide"
QMQLVQWGAGLLKPSETLSLTCAVYGGSFSGYYWSWIRQPPGKGLEWIGEINHSGSTNYNPSLKSRVTMSVDTSKHQFSLKLSSVTAADTAVYYCARWWELPDYWGQGTLVTVSS

SEQ ID NO: 27 - protein, 107 aa, synthetic construct
  REGION 1..107: note = source = /note="Description of Artificial Sequence: Synthetic polypeptide"
EIVLTQSPSSLSASVGDRVTITCRASQGIRNDLGWYQQKPGKAPKRLIYAASSLQSGVPSRFSGSGSGTEFTLTISSLQPEDFATYYCLQHNSYPWTFGQGTKVEIK

SEQ ID NO: 28 - protein, 8 aa, synthetic construct
  REGION 1..8: note = source = /note="Description of Artificial Sequence: Synthetic peptide"
GGSFSGYY

SEQ ID NO: 29 - protein, 7 aa, synthetic construct
  REGION 1..7: note = source = /note="Description of Artificial Sequence: Synthetic peptide"
INHSGST

SEQ ID NO: 30 - protein, 11 aa, synthetic construct
  REGION 1..11: note = source = /note="Description of Artificial Sequence: Synthetic peptide"
CARWWELPDYW

SEQ ID NO: 31 - protein, 6 aa, synthetic construct
  REGION 1..6: note = source = /note="Description of Artificial Sequence: Synthetic peptide"
QGIRND

SEQ ID NO: 32 - skipped

SEQ ID NO: 33 - protein, 11 aa, synthetic construct [sequence omitted]

SEQ ID NO: 34 - DNA, 351 bp, synthetic construct
  misc_feature 1..351: note = source = /note="Description of Artificial Sequence: Synthetic polynucleotide"
  source 1..351: mol_type = other DNA
cagatgcagctggtgcaatggggcgcaggactgttgaagccttcggagaccctgtccctcacctgcgctgtctatggtgggtccttcagtggttactactggagctggatccgccagcccccagggaaggggctggagtggattggggaaatcaatcatagtggaagcaccaactacaacccgtccctcaagagtcgagtcaccatatcagtagacacgtccaagaaccagttctccctgaagctgagctctgtgaccgccgcggacacggctgtgtattactgtgcgaggttttactatgctccgaactttgactactggggccagggcaccctggtcaccgtctcgagt

SEQ ID NO: 35 - DNA, 318 bp, synthetic construct
  misc_feature 1..318: note = source = /note="Description of Artificial Sequence: Synthetic polynucleotide"
  source 1..318: mol_type = other DNA
gaaattgtgttgacgcagtctccttccaccctgtctgcatctgtaggagacagagtcaccatcacttgccgggccagtcagagtattagtagctggttggcctggtatcagcagaaaccagggacagcccctaagctcctgatctataaggcgtctagtttagaaagtggggtcccatcaaggttcagcggcagtggatctgggacagaattcactctcaccatcagcagcctgcagcctgatgattttgcaacttattactgccaacagtataatagttattccactttcggcggagggaccaaggtggagatcaaa

SEQ ID NO: 36 - protein, 117 aa, synthetic construct
  REGION 1..117: note = source = /note="Description of Artificial Sequence: Synthetic polypeptide"
QMQLVQWGAGLLKPSETLSLTCAVYGGSFSGYYWSWIRQPPGKGLEWIGEINHSGSTNYNPSLKSRVTISVDTSKNQFSLKLSSVTAADTAVYYCARFYYAPNFDYWGQGTLVTVSS

SEQ ID NO: 37 - protein, 106 aa, synthetic construct
  REGION 1..106: note = source = /note="Description of Artificial Sequence: Synthetic polypeptide"
EIVLTQSPSTLSASVGDRVTITCRASQSISSWLAWYQQKPGTAPKLLIYKASSLESGVPSRFSGSGSGTEFTLTISSLQPDDFATYYCQQYNSYSTFGGGTKVEIK

SEQ ID NO: 38 - protein, 8 aa, synthetic construct
  REGION 1..8: note = source = /note="Description of Artificial Sequence: Synthetic peptide"
GGSFSGYY

SEQ ID NO: 39 - protein, 7 aa, synthetic construct
  REGION 1..7: note = source = /note="Description of Artificial Sequence: Synthetic peptide"
INHSGST

SEQ ID NO: 40 - protein, 13 aa, synthetic construct
  REGION 1..13: note = source = /note="Description of Artificial Sequence: Synthetic peptide"
CARFYYAPNFDYW

SEQ ID NO: 41 - protein, 6 aa, synthetic construct
  REGION 1..6: note = source = /note="Description of Artificial Sequence: Synthetic peptide"
QSISSW

SEQ ID NO: 42 - skipped

SEQ ID NO: 43 - protein, 10 aa, synthetic construct [sequence omitted]

SEQ ID NO: 44 - DNA, 360 bp, synthetic construct
  misc_feature 1..360: note = source = /note="Description of Artificial Sequence: Synthetic polynucleotide"
  source 1..360: mol_type = other DNA
caggtgcagctgcagcagtcgggcccaggactggtgaagccttcggagaccctgtccctcacctgcactgtctctggtggctccatcagcagtagtaattactactggggctggatccgccagcccccagggaaggggctggagtggattgggagtatctattatagtgggaacacctactacaacccgtccctcaagagtcgagtcaccatatccgtagacacgtccaagaaccagttctccctgaagctgagttctgtgaccgccgcagacacggctgtgtattactgtgcgagacagacagtggctggccccctctttgactactggggccagggaaccctggtcaccgtctcgagt

SEQ ID NO: 45 - DNA, 321 bp, synthetic construct
  misc_feature 1..321: note = source = /note="Description of Artificial Sequence: Synthetic polynucleotide"
  source 1..321: mol_type = other DNA
gaaattgtgatgacgcagtctccttccaccctgtctgcatctgtaggagacagagtcaccatcacttgccgggccagtcagagtattagtagctggttggcctggtatcagcagaaaccagggaaagcccctaaggtcctgatctataaggcgtctagtttagaaagtggggtcccatcaaggttcagcggcagtggatctgggacagaactcactctcaccatcagcagcctgcagcctgatgattttgcaacttattactgccaacagtataatagttattcattcactttcggccctgggaccaaagtggatatcaag

SEQ ID NO: 46 - protein, 120 aa, synthetic construct
  REGION 1..120: note = source = /note="Description of Artificial Sequence: Synthetic polypeptide"
QVQLQQSGPGLVKPSETLSLTCTVSGGSISSSNYYWGWIRQPPGKGLEWIGSIYYSGNTYYNPSLKSRVTISVDTSKNQFSLKLSSVTAADTAVYYCARQTVAGPLFDYWGQGTLVTVSS

SEQ ID NO: 47 - protein, 107 aa, synthetic construct
  REGION 1..107: note = source = /note="Description of Artificial Sequence: Synthetic polypeptide"
EIVMTQSPSTLSASVGDRVTITCRASQSISSWLAWYQQKPGKAPKVLIYKASSLESGVPSRFSGSGSGTELTLTISSLQPDDFATYYCQQYNSYSFTFGPGTKVDIK

SEQ ID NO: 48 - protein, 10 aa, synthetic construct
  REGION 1..10: note = source = /note="Description of Artificial Sequence: Synthetic peptide"
GGSISSSNYY

SEQ ID NO: 49 - protein, 7 aa, synthetic construct
  REGION 1..7: note = source = /note="Description of Artificial Sequence: Synthetic peptide"
IYYSGNT

SEQ ID NO: 50 - protein, 14 aa, synthetic construct
  REGION 1..14: note = source = /note="Description of Artificial Sequence: Synthetic peptide"
CARQTVAGPLFDYW

SEQ ID NO: 51 - protein, 6 aa, synthetic construct
  REGION 1..6: note = source = /note="Description of Artificial Sequence: Synthetic peptide"
QSISSW

SEQ ID NO: 52 - skipped

SEQ ID NO: 53 - protein, 11 aa, synthetic construct [sequence omitted]

SEQ ID NO: 54 - DNA, 375 bp, synthetic construct
  misc_feature 1..375: note = source = /note="Description of Artificial Sequence: Synthetic polynucleotide"
  source 1..375: mol_type = other DNA
caggtccagctggtgcaatctggggctgaggtgaagaagcctggggcctcagtgaaggtctcctgcaaggctgctggatacaccttaaccggctactatatgcactgggtgcgacaggcccctggacaaggccttgagtggatgggacggatcaaccctaacagtggtggctcaaacaatgcacagaagtttcagggcagggtcaccatgaccagggacacgtccatcagcacagcctacatggagctgagcaggctgagatctgacgacacggccgtgtattactgtgcgagagagggtcccctgtatagcagtggctggtacgagggtgcttttgatatctggggccaagggacaatggtcaccgtctcgagt

SEQ ID NO: 55 - DNA, 327 bp, synthetic construct
  misc_feature 1..327: note = source = /note="Description of Artificial Sequence: Synthetic polynucleotide"
  source 1..327: mol_type = other DNA
gaaattgtgatgacgcagtctccttccaccctgtctgcatctgtaggagacagagtcaccatcacttgccgggccagtcagagtattagtagttggttggcctggtatcagcagaaaccagggaaagcccctaagctcctgatctataaggcgtctagtttagaaagtggggtcccatcaaggttcagcggcagtggatctgggacagaattcactctcaccatcagcagcctgcagcctgatgattttgcaacttattactgccaacagtataatagttattctccggggctcactttcggcggagggaccaaggtggagatcaag

SEQ ID NO: 56 - protein, 125 aa, synthetic construct
  REGION 1..125: note = source = /note="Description of Artificial Sequence: Synthetic polypeptide"
QVQLVQSGAEVKKPGASVKVSCKAAGYTLTGYYMHWVRQAPGQGLEWMGRINPNSGGSNNAQKFQGRVTMTRDTSISTAYMELSRLRSDDTAVYYCAREGPLYSSGWYEGAFDIWGQGTMVTVSS

SEQ ID NO: 57 - protein, 109 aa, synthetic construct
  REGION 1..109: note = source = /note="Description of Artificial Sequence: Synthetic polypeptide"
EIVMTQSPSTLSASVGDRVTITCRASQSISSWLAWYQQKPGKAPKLLIYKASSLESGVPSRFSGSGSGTEFTLTISSLQPDDFATYYCQQYNSYSPGLTFGGGTKVEIK

SEQ ID NO: 58 - protein, 8 aa, synthetic construct
  REGION 1..8: note = source = /note="Description of Artificial Sequence: Synthetic peptide"
GYTLTGYY

SEQ ID NO: 59 - protein, 8 aa, synthetic construct
  REGION 1..8: note = source = /note="Description of Artificial Sequence: Synthetic peptide"
INPNSGGS

SEQ ID NO: 60 - protein, 20 aa, synthetic construct
  REGION 1..20: note = source = /note="Description of Artificial Sequence: Synthetic peptide"
CAREGPLYSSGWYEGAFDIW

SEQ ID NO: 61 - protein, 6 aa, synthetic construct
  REGION 1..6: note = source = /note="Description of Artificial Sequence: Synthetic peptide"
QSISSW

SEQ ID NO: 62 - skipped

SEQ ID NO: 63 - protein, 13 aa, synthetic construct [sequence omitted]

SEQ ID NO: 64 - DNA, 372 bp, synthetic construct
  misc_feature 1..372: note = source = /note="Description of Artificial Sequence: Synthetic polynucleotide"
  source 1..372: mol_type = other DNA
cagatgcagctacagcagtcaggtccaggactggtgaagccctcgcagaccctctcactcacctgtgccatctccggggacagtgtctctagcaacagtgctgcttggaactggatcaggcagtccccatcgagaggccttgagtggctgggaaggacatactacaggtccaagtggtattctgcttttgcagtatctgtgaaaagtcgaataaccatcaacccagacacatccaagaaccagttctccctgcagctgaactctgtgactcccgaggacacggctgtgtattactgtgcaagagagggtagcagtggctggtacggatacgtccaccactggggccagggcaccctggtcaccgtctcgagt

SEQ ID NO: 65 - DNA, 321 bp, synthetic construct
  misc_feature 1..321: note = source = /note="Description of Artificial Sequence: Synthetic polynucleotide"
  source 1..321: mol_type = other DNA
gaaattgtgttgacgcagtctccagcttccctgtctgtatctctgggagaaactgtcaccatcgaatgtcgagcaagtgaggacatttacaatggtttagcatggtatcagcagaagccagggaaatctcctcagctcctgatctataatgcaaatagcttgcatactggggtcccatcacggttcagtggcagtggatctggtacacagtattctctcaagataaacagcctgcaatctgaagatgtcgcaagttatttctgtcaacagtattacgattatcctccgacgttcggccaagggaccaaggtggaaatcaaa

SEQ ID NO: 66 - protein, 124 aa, synthetic construct
  REGION 1..124: note = source = /note="Description of Artificial Sequence: Synthetic polypeptide"
QMQLQQSGPGLVKPSQTLSLTCAISGDSVSSNSAAWNWIRQSPSRGLEWLGRTYYRSKWYSAFAVSVKSRITINPDTSKNQFSLQLNSVTPEDTAVYYCAREGSSGWYGYVHHWGQGTLVTVSS

SEQ ID NO: 67 - protein, 107 aa, synthetic construct
  REGION 1..107: note = source = /note="Description of Artificial Sequence: Synthetic polypeptide"
EIVLTQSPASLSVSLGETVTIECRASEDIYNGLAWYQQKPGKSPQLLIYNANSLHTGVPSRFSGSGSGTQYSLKINSLQSEDVASYFCQQYYDYPPTFGQGTKVEIK

SEQ ID NO: 68 - protein, 10 aa, synthetic construct
  REGION 1..10: note = source = /note="Description of Artificial Sequence: Synthetic peptide"
GDSVSSNSAA

SEQ ID NO: 69 - protein, 9 aa, synthetic construct
  REGION 1..9: note = source = /note="Description of Artificial Sequence: Synthetic peptide"
TYYRSKWYS

SEQ ID NO: 70 - protein, 16 aa, synthetic construct
  REGION 1..16: note = source = /note="Description of Artificial Sequence: Synthetic peptide"
CAREGSSGWYGYVHHW

SEQ ID NO: 71 - protein, 6 aa, synthetic construct
  REGION 1..6: note = source = /note="Description of Artificial Sequence: Synthetic peptide"
EDIYNG

SEQ ID NO: 72 - skipped

SEQ ID NO: 73 - protein, 11 aa, synthetic construct
  REGION 1..11: note = source = /note="Description of Artificial Sequence: Synthetic peptide"
CQQYYDYPPTF

SEQ ID NO: 74 - DNA, 369 bp, synthetic construct
  misc_feature 1..369: note = source = /note="Description of Artificial Sequence: Synthetic polynucleotide"
  source 1..369: mol_type = other DNA
caggtgcagctgcaggagtcgggcccaggactggtgaagccttcggagaccctgtccctcacctgcactgtctctggtggctccttcagcagtagtagttactactggggctggatccgccagccccctgggaaggggctggagtggattgggatcttctattatagtgggaccacctactacaacccgtccctcaagagtcgagtcaccatatccgcacacacgtccaagagccagttctccctgaagctgagctctgtgaccgccgcagacacggctgtgtattactgtgcgagagggggagaatattttgaccggttactcccctttgactactggggccagggaaccctggtcaccgtctcgagt

SEQ ID NO: 75 - DNA, 321 bp, synthetic construct
  misc_feature 1..321: note = source = /note="Description of Artificial Sequence: Synthetic polynucleotide"
  source 1..321: mol_type = other DNA
gaaattgtgatgacgcagtctccatccttcctgtctgcatctgtaggagacagagtcaccatcacttgccgggccagtcagggcattagcagttatttagcctggtatcagcaaaaaccagggaaagcccctaagctcctgatctatgctgcatccactttggaaagtggggtcccatcaaggttcagcggcagtggatctgggacagaattcactctcacaatcagcagcctgcagcctgaagattttgcaacttattactgtcaacagcttaatagttacccattcactttcggccctgggaccaaagtggatatcaaa

SEQ ID NO: 76 - protein, 123 aa, synthetic construct
  REGION 1..123: note = source = /note="Description of Artificial Sequence: Synthetic polypeptide"
QVQLQESGPGLVKPSETLSLTCTVSGGSFSSSSYYWGWIRQPPGKGLEWIGIFYYSGTTYYNPSLKSRVTISAHTSKSQFSLKLSSVTAADTAVYYCARGGEYFDRLLPFDYWGQGTLVTVSS

SEQ ID NO: 77 - protein, 107 aa, synthetic construct
  REGION 1..107: note = source = /note="Description of Artificial Sequence: Synthetic polypeptide"
EIVMTQSPSFLSASVGDRVTITCRASQGISSYLAWYQQKPGKAPKLLIYAASTLESGVPSRFSGSGSGTEFTLTISSLQPEDFATYYCQQLNSYPFTFGPGTKVDIK

SEQ ID NO: 78 - protein, 10 aa, synthetic construct
  REGION 1..10: note = source = /note="Description of Artificial Sequence: Synthetic peptide"
GGSFSSSSYY

SEQ ID NO: 79 - protein, 7 aa, synthetic construct
  REGION 1..7: note = source = /note="Description of Artificial Sequence: Synthetic peptide"
FYYSGTT

SEQ ID NO: 80 - protein, 17 aa, synthetic construct
  REGION 1..17: note = source = /note="Description of Artificial Sequence: Synthetic peptide"
CARGGEYFDRLLPFDYW

SEQ ID NO: 81 - protein, 6 aa, synthetic construct
  REGION 1..6: note = source = /note="Description of Artificial Sequence: Synthetic peptide"
QGISSY

SEQ ID NO: 82 - skipped

SEQ ID NO: 83 - protein, 11 aa, synthetic construct [sequence omitted]

SEQ ID NO: 84 - DNA, 351 bp, synthetic construct
  misc_feature 1..351: note = source = /note="Description of Artificial Sequence: Synthetic polynucleotide"
  source 1..351: mol_type = other DNA
caggtgcagctggtggagtctgggggaggcttggtacagccgggggggtccctgagactctcctgtacagcctctggattcacctttagcagctatgccatgagctgggtccgccaggctccagggaaggggctggagtgggtctcagctattggtggtagtggtggtagcacatactacgcagactccgtgaagggccggttcaccatctccagagacaattccaagaacacgctgtatctgcaaatgaacagcctgagagccgaggacacggccgtatattactgtgtgaaagatggggcaggaggctttgactactggggccagggaaccctggtcaccgtctcgagt

SEQ ID NO: 85 - DNA, 321 bp, synthetic construct
  misc_feature 1..321: note = source = /note="Description of Artificial Sequence: Synthetic polynucleotide"
  source 1..321: mol_type = other DNA
gatattgtgatgacgcagtcttcatcctccctgtctgcatctgtaggagacagagtcaccatcacttgccgggcaagtcagggcattataaatcatttaggctggtatcagcataaaccagggaaagcccctaatcgcctaatctatgctgcatccagtttgcaaagtggggtcccatcaaggttcagcggcagtggatctgggacagaattcactctcacaatcagcagcctgcagcctgaagattttgcaacttattactgtctacggcataatagttaccctccgacgttcggccaagggaccaaggtggaaatcaag

SEQ ID NO: 86 - protein, 117 aa, synthetic construct
  REGION 1..117: note = source = /note="Description of Artificial Sequence: Synthetic polypeptide"
QVQLVESGGGLVQPGGSLRLSCTASGFTFSSYAMSWVRQAPGKGLEWVSAIGGSGGSTYYADSVKGRFTISRDNSKNTLYLQMNSLRAEDTAVYYCVKDGAGGFDYWGQGTLVTVSS

SEQ ID NO: 87 - protein, 107 aa, synthetic construct
  REGION 1..107: note = source = /note="Description of Artificial Sequence: Synthetic polypeptide"
DIVMTQSSSSLSASVGDRVTITCRASQGIINHLGWYQHKPGKAPNRLIYAASSLQSGVPSRFSGSGSGTEFTLTISSLQPEDFATYYCLRHNSYPPTFGQGTKVEIK

SEQ ID NO: 88 - protein, 8 aa, synthetic construct
  REGION 1..8: note = source = /note="Description of Artificial Sequence: Synthetic peptide"
GFTFSSYA

SEQ ID NO: 89 - protein, 8 aa, synthetic construct
  REGION 1..8: note = source = /note="Description of Artificial Sequence: Synthetic peptide"
IGGSGGST

SEQ ID NO: 90 - protein, 12 aa, synthetic construct
  REGION 1..12: note = source = /note="Description of Artificial Sequence: Synthetic peptide"
CVKDGAGGFDYW

SEQ ID NO: 91 - protein, 6 aa, synthetic construct
  REGION 1..6: note = source = /note="Description of Artificial Sequence: Synthetic peptide"
QGIINH

SEQ ID NO: 92 - skipped

SEQ ID NO: 93 - protein, 5 aa, synthetic construct
  REGION 1..5: note = source = /note="Description of Artificial Sequence: Synthetic peptide"
YPPTF

SEQ ID NO: 94 - DNA, 366 bp, synthetic construct
  misc_feature 1..366: note = source = /note="Description of Artificial Sequence: Synthetic polynucleotide"
  source 1..366: mol_type = other DNA
caggtgcagctacagcagtcgggcccaggactggtgaagccttcacagaccctgtccctcacctgcactgtctctggtggctccatcaacagtggtggtcactactggagctggatccgccagcacccagggaggggcctggagtggattgggtacatctattacagtgggagcatctactacaacccgtccctcaagagtcgacttaccatatcagtagacacgtctaagaaccagttctccctgaagctgagctctgtgactgccgcggacacggccgtgtattactgtgcgagttattactatgccagtagtggtgatgcttttgatatctggggccaagggacaatggtcaccgtctcgagt

SEQ ID NO: 95 - DNA, 321 bp, synthetic construct
  misc_feature 1..321: note = source = /note="Description of Artificial Sequence: Synthetic polynucleotide"
  source 1..321: mol_type = other DNA
gaaacgacactcacgcagtctccagccaccctgtctttgtctccaggggaaagagccaccctctcctgcagggccagtcagagtgttagcagctacttagcctggtaccaacagaaacctggccaggctcccaggctcctcatctatgatgcatccaacagggccactggcatcccagccaggttcagtggcagtgggtctgggacagacttcactctcaccatcagcagcctagagcctgaagattttgcagtttattactgtcagcagcgtagcaactggcctccgacgttcggccaagggaccaaggtggaaatcaaa

SEQ ID NO: 96 - protein, 122 aa, synthetic construct
  REGION 1..122: note = source = /note="Description of Artificial Sequence: Synthetic polypeptide"
QVQLQQSGPGLVKPSQTLSLTCTVSGGSINSGGHYWSWIRQHPGRGLEWIGYIYYSGSIYYNPSLKSRLTISVDTSKNQFSLKLSSVTAADTAVYYCASYYYASSGDAFDIWGQGTMVTVSS

SEQ ID NO: 97 - protein, 107 aa, synthetic construct
  REGION 1..107: note = source = /note="Description of Artificial Sequence: Synthetic polypeptide"
ETTLTQSPATLSLSPGERATLSCRASQSVSSYLAWYQQKPGQAPRLLIYDASNRATGIPARFSGSGSGTDFTLTISSLEPEDFAVYYCQQRSNWPPTFGQGTKVEIK

SEQ ID NO: 98 - protein, 10 aa, synthetic construct
  REGION 1..10: note = source = /note="Description of Artificial Sequence: Synthetic peptide"
GGSINSGGHY

SEQ ID NO: 99 - protein, 7 aa, synthetic construct
  REGION 1..7: note = source = /note="Description of Artificial Sequence: Synthetic peptide"
IYYSGSI

SEQ ID NO: 100 - protein, 16 aa, synthetic construct
  REGION 1..16: note = source = /note="Description of Artificial Sequence: Synthetic peptide"
CASYYYASSGDAFDIW

SEQ ID NO: 101 - protein, 6 aa, synthetic construct
  REGION 1..6: note = source = /note="Description of Artificial Sequence: Synthetic peptide"
QSVSSY

SEQ ID NO: 102 - skipped

SEQ ID NO: 103 - protein, 11 aa, synthetic construct [sequence omitted]

SEQ ID NO: 104 - DNA, 372 bp, synthetic construct
  misc_feature 1..372: note = source = /note="Description of Artificial Sequence: Synthetic polynucleotide"
  source 1..372: mol_type = other DNA
caggtgcagctgcaggagtctgggggaggcttggtacagccgggggggtccctgagactctcctgtacagcctctggattcacctttagtaattatgccatgagctgggtccgccaggctccagggaaggggctggagtgggtctcagctattagtggtcgtggtggtagcacattcttcgcagactccgtgaagggccggttcaccatctccagagacaattccaagagcacgctgtatctgcaaacgaacagcctgagagccgaggacacggccgtatattactgtgcgaaagggggcccgttgtataactggaacgacggtgatggttttgatatctggggccaagggaccacggtcacagtctcgagt

SEQ ID NO: 105 - DNA, 324 bp, synthetic construct
  misc_feature 1..324: note = source = /note="Description of Artificial Sequence: Synthetic polynucleotide"
  source 1..324: mol_type = other DNA
gaaattgtgttgacgcagtctccagccaccctgtctgtgtctccaggggaaagagccaccctctcctgcagggccagtcagagtgttagcagcaacttagcctggtaccagcagaaacctggccaggctcccaggctcctcatctatggtgcatccaccagggccactggtatcccagccaggttcagtggcactgggtctgggacagagttcactctcaccatcagcagcctgcagtctgaagattttgcactttattactgtcagcagtatgataactggcctccgtggacgttcggccaagggaccaaggtggaaatcaaa

SEQ ID NO: 106 - protein, 124 aa, synthetic construct
  REGION 1..124: note = source = /note="Description of Artificial Sequence: Synthetic polypeptide"
QVQLQESGGGLVQPGGSLRLSCTASGFTFSNYAMSWVRQAPGKGLEWVSAISGRGGSTFFADSVKGRFTISRDNSKSTLYLQTNSLRAEDTAVYYCAKGGPLYNWNDGDGFDIWGQGTTVTVSS

SEQ ID NO: 107 - protein, 108 aa, synthetic construct
  REGION 1..108: note = source = /note="Description of Artificial Sequence: Synthetic polypeptide"
EIVLTQSPATLSVSPGERATLSCRASQSVSSNLAWYQQKPGQAPRLLIYGASTRATGIPARFSGTGSGTEFTLTISSLQSEDFALYYCQQYDNWPPWTFGQGTKVEIK

SEQ ID NO: 108 - protein, 8 aa, synthetic construct
  REGION 1..8: note = source = /note="Description of Artificial Sequence: Synthetic peptide"
GFTFSNYA

SEQ ID NO: 109 - protein, 8 aa, synthetic construct
  REGION 1..8: note = source = /note="Description of Artificial Sequence: Synthetic peptide"
ISGRGGST

SEQ ID NO: 110 - protein, 19 aa, synthetic construct
  REGION 1..19: note = source = /note="Description of Artificial Sequence: Synthetic peptide"
CAKGGPLYNWNDGDGFDIW

SEQ ID NO: 111 - protein, 6 aa, synthetic construct
  REGION 1..6: note = source = /note="Description of Artificial Sequence: Synthetic peptide"
QSVSSN

SEQ ID NO: 112 - skipped

SEQ ID NO: 113 - protein, 12 aa, synthetic construct [sequence omitted]

SEQ ID NO: 114 - DNA, 357 bp, synthetic construct
  misc_feature 1..357: note = source = /note="Description of Artificial Sequence: Synthetic polynucleotide"
  source 1..357: mol_type = other DNA
caggtgcagctgcaggagtctgggggaggcttggtcaagcctggagggtccctgagactctcctgtgcagcctctggattcaccttcagtgactactacatgacctggatccgccaggctccagggaaggggctggagtggatttcatacattagtggtggtggtggttccatatactacgcagactctgtgaagggccgattcaccatctccagggacaacgccaagaactcactgtatctgcaaatgaacagcctgagagccgaggacacggccgtttatttctgtgcgagagggaactggggatcggcggctcttgatatctggggccaagggacaatggtcacggtctcgagt

SEQ ID NO: 115 - DNA, 321 bp, synthetic construct
  misc_feature 1..321: note = source = /note="Description of Artificial Sequence: Synthetic polynucleotide"
  source 1..321: mol_type = other DNA
gaaattgtgttgacgcagtctccatcctcactgtctgcatctgtaggagacagagtcaccatcacttgtcgggcgagtcagggcattaacaattatttagcctggtttcagcagaaaccagggagagcccctaagtccctgatctatgctgcatccagtttgcaaagtggggtcccatcgaagttcagcggcagtggatctgggacagatttcactctcaccatcagcagcctgcagcctgaagattttgcaacttattactgccaacagtataatagttaccctccaactctcggccctgggaccaacgtggatatcaaa

SEQ ID NO: 116 - protein, 119 aa, synthetic construct
  REGION 1..119: note = source = /note="Description of Artificial Sequence: Synthetic polypeptide"
QVQLQESGGGLVKPGGSLRLSCAASGFTFSDYYMTWIRQAPGKGLEWISYISGGGGSIYYADSVKGRFTISRDNAKNSLYLQMNSLRAEDTAVYFCARGNWGSAALDIWGQGTMVTVSS

SEQ ID NO: 117 - protein, 107 aa, synthetic construct
  REGION 1..107: note = source = /note="Description of Artificial Sequence: Synthetic polypeptide"
EIVLTQSPSSLSASVGDRVTITCRASQGINNYLAWFQQKPGRAPKSLIYAASSLQSGVPSKFSGSGSGTDFTLTISSLQPEDFATYYCQQYNSYPPTLGPGTNVDIK

SEQ ID NO: 118 - protein, 8 aa, synthetic construct
  REGION 1..8: note = source = /note="Description of Artificial Sequence: Synthetic peptide"
GFTFSDYY

SEQ ID NO: 119 - protein, 11 aa, synthetic construct
  REGION 1..11: note = source = /note="Description of Artificial Sequence: Synthetic peptide"
ISYISGGGGSI

SEQ ID NO: 120 - protein, 14 aa, synthetic construct
  REGION 1..14: note = source = /note="Description of Artificial Sequence: Synthetic peptide"
CARGNWGSAALDIW

SEQ ID NO: 121 - protein, 6 aa, synthetic construct
  REGION 1..6: note = source = /note="Description of Artificial Sequence: Synthetic peptide"
QGINNY

SEQ ID NO: 122 - skipped

SEQ ID NO: 123 - protein, 11 aa, synthetic construct
  REGION 1..11: note = source = /note="Description of Artificial Sequence: Synthetic peptide"
CQQYNSYPPTL

SEQ ID NO: 124 - DNA, 351 bp, synthetic construct
  misc_feature 1..351: note = source = /note="Description of Artificial Sequence: Synthetic polynucleotide"
  source 1..351: mol_type = other DNA
caggtgcagctggtggagtctgggggaggcttggtacagccgggggggtccctgagactctcctgtacagcctctggattcacctttagcagctatgccatgagctgggtccgccaggctccagggaaggggctggagtgggtctcagctattggtggtagtggtggtagcgcatactacgcagactccgtgaagggccggttcaccatctccagagacaattccaagaacacgctgtatctgcaaatgaacagcctgagagccgaggacacggccgtatattactgtgtgaaagatggggcaggaggctttgactactggggccagggcaccctggtcaccgtctcgagt

SEQ ID NO: 125 - DNA, 321 bp, synthetic construct
  misc_feature 1..321: note = source = /note="Description of Artificial Sequence: Synthetic polynucleotide"
  source 1..321: mol_type = other DNA
gacatccagttgacccagtccccatcctccctgtctgcatctgtaggagacagagtcaccatcacttgccgggcaagtcagggcattagaaatcatttaggctggtatcagcagaaaccagggaaagcccctaagcgcctaatctatgctgcatccagtttgcaaagtggggtcccatcaaggttcagcggcagtggatctgggacagaattcactctcacaatcagcagcctgcagcctgaagattttgcaacttattactgtctacagcataatagttaccctccgacgttcggccaagggaccaaggtggaaatcaag

SEQ ID NO: 126 - protein, 117 aa, synthetic construct
  REGION 1..117: note = source = /note="Description of Artificial Sequence: Synthetic polypeptide"
QVQLVESGGGLVQPGGSLRLSCTASGFTFSSYAMSWVRQAPGKGLEWVSAIGGSGGSAYYADSVKGRFTISRDNSKNTLYLQMNSLRAEDTAVYYCVKDGAGGFDYWGQGTLVTVSS

SEQ ID NO: 127 - protein, 107 aa, synthetic construct
  REGION 1..107: note = source = /note="Description of Artificial Sequence: Synthetic polypeptide"
DIQLTQSPSSLSASVGDRVTITCRASQGIRNHLGWYQQKPGKAPKRLIYAASSLQSGVPSRFSGSGSGTEFTLTISSLQPEDFATYYCLQHNSYPPTFGQGTKVEIK

SEQ ID NO: 128 - protein, 8 aa, synthetic construct
  REGION 1..8: note = source = /note="Description of Artificial Sequence: Synthetic peptide"
GFTFSSYA

SEQ ID NO: 129 - protein, 8 aa, synthetic construct
  REGION 1..8: note = source = /note="Description of Artificial Sequence: Synthetic peptide"
IGGSGGSA

SEQ ID NO: 130 - protein, 12 aa, synthetic construct
  REGION 1..12: note = source = /note="Description of Artificial Sequence: Synthetic peptide"
CVKDGAGGFDYW

SEQ ID NO: 131 - protein, 6 aa, synthetic construct
  REGION 1..6: note = source = /note="Description of Artificial Sequence: Synthetic peptide"
QGIRNH

SEQ ID NO: 132 - skipped

SEQ ID NO: 133 - protein, 11 aa, synthetic construct [sequence omitted]

SEQ ID NO: 134 - DNA, 354 bp, synthetic construct
  misc_feature 1..354: note = source = /note="Description of Artificial Sequence: Synthetic polynucleotide"
  source 1..354: mol_type = other DNA
cagatgcagctacagcagtctgggggaggcttggtacagccgggggggtccctgagactctcctgtgcagcctctggattcaccgttagcagctatgccatgagctgggtccgccaggctctagggaaggggctggagtgggtctcaggtattagtggtagtggtggtagcacatactacgcagactccgtgaagggccggttcaccatctccagagacaattccaagaatacgctgtatctgcaaatgaacagcctgagagccgaggacacggccgtatattactgtgcgaagatagtgggagctacccactttgactactggggccagggaaccctggtcacggtctcgagt

SEQ ID NO: 135 - DNA, 339 bp, synthetic construct
  misc_feature 1..339: note = source = /note="Description of Artificial Sequence: Synthetic polynucleotide"
  source 1..339: mol_type = other DNA
gaaattgtgatgacacagtctccagactccctggctgtgtctctgggcgagagggccaccatcaactgcaagtccagccagagtgttttatacagctccaacaataagaactacttagcttggtaccagcagaaaccaggacagcctcctaagctgctcatttactgggcatctacccgggaatccggggtccctgaccgattcagtggcagcgggtctgggacagatttcactctcaccatcagcagcctgcaggctgaagatgtggcagtttattactgtcagcaatattatagtggtccgatcaccttcggccaagggacacgactggagattaag

SEQ ID NO: 136 - protein, 118 aa, synthetic construct
  REGION 1..118: note = source = /note="Description of Artificial Sequence: Synthetic polypeptide"
QMQLQQSGGGLVQPGGSLRLSCAASGFTVSSYAMSWVRQALGKGLEWVSGISGSGGSTYYADSVKGRFTISRDNSKNTLYLQMNSLRAEDTAVYYCAKIVGATHFDYWGQGTLVTVSS

SEQ ID NO: 137 - protein, 113 aa, synthetic construct
  REGION 1..113: note = source = /note="Description of Artificial Sequence: Synthetic polypeptide"
EIVMTQSPDSLAVSLGERATINCKSSQSVLYSSNNKNYLAWYQQKPGQPPKLLIYWASTRESGVPDRFSGSGSGTDFTLTISSLQAEDVAVYYCQQYYSGPITFGQGTRLEIK

SEQ ID NO: 138 - protein, 8 aa, synthetic construct
  REGION 1..8: note = source = /note="Description of Artificial Sequence: Synthetic peptide"
GFTVSSYA

SEQ ID NO: 139 - protein, 8 aa, synthetic construct
  REGION 1..8: note = source = /note="Description of Artificial Sequence: Synthetic peptide"
ISGSGGST

SEQ ID NO: 140 - protein, 13 aa, synthetic construct
  REGION 1..13: note = source = /note="Description of Artificial Sequence: Synthetic peptide"
CAKIVGATHFDYW

SEQ ID NO: 141 - protein, 12 aa, synthetic construct
  REGION 1..12: note = source = /note="Description of Artificial Sequence: Synthetic peptide"
QSVLYSSNNKNY

SEQ ID NO: 142 - skipped

SEQ ID NO: 143 - protein, 11 aa, synthetic construct [sequence omitted]

SEQ ID NO: 144 - DNA, 366 bp, synthetic construct
  misc_feature 1..366: note = source = /note="Description of Artificial Sequence: Synthetic polynucleotide"
  source 1..366: mol_type = other DNA
caggtgcagctggtggagtcgggcccaggactggtgaagccttcacagaccctgtccctcacctgcactgtctctggtggctccatcaacagtggtggttactactggagctggatccgccagcacccagggaagggcctggagtggattgggtacatctattacagtgggagcatctactacaacccgtccctcaggagtcgacttaccatatcagtagacacgtctaagaaccagttctccctgaagctgagctctgtgactgccgcggacacggccgtttattactgtgcgactccttattactatggttcggggagttatggggactactggggccagggcaccctggtcactgtctcgagt

SEQ ID NO: 145 - DNA, 321 bp, synthetic construct
  misc_feature 1..321: note = source = /note="Description of Artificial Sequence: Synthetic polynucleotide"
  source 1..321: mol_type = other DNA
gacatccagatgacccagtctccagccaccctgtctttgtctccaggggaaagagccaccctctcctgcagggccagtcagagtgttaacaactacttagcctggtaccaacagaaacctggccaggctcccaggctcctcatctatgatgcatccaacagggccactggcatcccagccaggttcagtggcagtgggtctgggacagacttcactctcaccatcagcagcctagagcctgaagattttgcagtttattactgtcagcagcgtagcaactggcccatcaccttcggccaagggacacgactggagattaaa

SEQ ID NO: 146 - protein, 122 aa, synthetic construct
  REGION 1..122: note = source = /note="Description of Artificial Sequence: Synthetic polypeptide"
QVQLVESGPGLVKPSQTLSLTCTVSGGSINSGGYYWSWIRQHPGKGLEWIGYIYYSGSIYYNPSLRSRLTISVDTSKNQFSLKLSSVTAADTAVYYCATPYYYGSGSYGDYWGQGTLVTVSS

SEQ ID NO: 147 - protein, 107 aa, synthetic construct
  REGION 1..107: note = source = /note="Description of Artificial Sequence: Synthetic polypeptide"
DIQMTQSPATLSLSPGERATLSCRASQSVNNYLAWYQQKPGQAPRLLIYDASNRATGIPARFSGSGSGTDFTLTISSLEPEDFAVYYCQQRSNWPITFGQGTRLEIK

SEQ ID NO: 148 - protein, 10 aa, synthetic construct
  REGION 1..10: note = source = /note="Description of Artificial Sequence: Synthetic peptide"
GGSINSGGYY

SEQ ID NO: 149 - protein, 7 aa, synthetic construct
  REGION 1..7: note = source = /note="Description of Artificial Sequence: Synthetic peptide"
IYYSGSI

SEQ ID NO: 150 - protein, 16 aa, synthetic construct
  REGION 1..16: note = source = /note="Description of Artificial Sequence: Synthetic peptide"
CATPYYYGSGSYGDYW

SEQ ID NO: 151 - protein, 6 aa, synthetic construct
  REGION 1..6: note = source = /note="Description of Artificial Sequence: Synthetic peptide"
QSVNNY

SEQ ID NO: 152 - skipped

SEQ ID NO: 153 - protein, 11 aa, synthetic construct [sequence omitted]

SEQ ID NO: 154 - DNA, 363 bp, synthetic construct
  misc_feature 1..363: note = source = /note="Description of Artificial Sequence: Synthetic polynucleotide"
  source 1..363: mol_type = other DNA
cagatgcagctgcaggagtcgggcccaggactggtgaagccttctcagaccctgtccctcacctgcactgtgtctggtggctccatcagcagtgttggttactactggaactggatccgccagcacccagggaagggcctggagttcattgggtacatctattacagtgggagcatctactacaatccgtccctcaagagtcgagttaccatatccgtagacacgtctaagaaccagttctccctgaagctgagctctgtgactgccgcggacacggccctatattactgtgcgagcgtcggtatagtgggagcctcctactttgagtactggggccagggaaccctggtcacagtctcgagt

SEQ ID NO: 155 - DNA, 321 bp, synthetic construct
  misc_feature 1..321: note = source = /note="Description of Artificial Sequence: Synthetic polynucleotide"
  source 1..321: mol_type = other DNA
gaaattgtgatgacacagtctccagccaccctgtctttgtctccaggggaaagagccaccctctcctgcagggccagtcagagtgttagcagctacttagcctggtaccaacagaaacctggccaggctcccaggctcctcatctatgatgcatccaacagggccactggcatcccagccaggttcagtggcagtgggtctgggacagacttcactctcaccatcagcagcctagagcctgaagattttgcagtttattactgtcagcagcgtagcaactggcctatcaccttcggccaagggacacgactggagatcaag

SEQ ID NO: 156 - protein, 121 aa, synthetic construct
  REGION 1..121: note = source = /note="Description of Artificial Sequence: Synthetic polypeptide"
QMQLQESGPGLVKPSQTLSLTCTVSGGSISSVGYYWNWIRQHPGKGLEFIGYIYYSGSIYYNPSLKSRVTISVDTSKNQFSLKLSSVTAADTALYYCASVGIVGASYFEYWGQGTLVTVSS

SEQ ID NO: 157 - protein, 107 aa, synthetic construct
  REGION 1..107: note = source = /note="Description of Artificial Sequence: Synthetic polypeptide"
EIVMTQSPATLSLSPGERATLSCRASQSVSSYLAWYQQKPGQAPRLLIYDASNRATGIPARFSGSGSGTDFTLTISSLEPEDFAVYYCQQRSNWPITFGQGTRLEIK

SEQ ID NO: 158 - protein, 10 aa, synthetic construct
  REGION 1..10: note = source = /note="Description of Artificial Sequence: Synthetic peptide"
GGSISSVGYY

SEQ ID NO: 159 - protein, 7 aa, synthetic construct
  REGION 1..7: note = source = /note="Description of Artificial Sequence: Synthetic peptide"
IYYSGSI

SEQ ID NO: 160 - protein, 15 aa, synthetic construct
  REGION 1..15: note = source = /note="Description of Artificial Sequence: Synthetic peptide"
CASVGIVGASYFEYW

SEQ ID NO: 161 - protein, 6 aa, synthetic construct
  REGION 1..6: note = source = /note="Description of Artificial Sequence: Synthetic peptide"
QSVSSY

SEQ ID NO: 162 - skipped

SEQ ID NO: 163 - protein, 11 aa, synthetic construct [sequence omitted]

SEQ ID NO: 164 - DNA, 354 bp, synthetic construct
  misc_feature 1..354: note = source = /note="Description of Artificial Sequence: Synthetic polynucleotide"
  source 1..354: mol_type = other DNA
caggtgcagctacagcagtctgggggaggcttggtacagcctggggggtccctgagactctcctgtgcagcctctggattcaccttaagcagctatgccatgagctgggtccgccaggctccagggaaggggctggagtgggtctcaggtattagtggtagtggtggtagcacatacaacgcagactccgtgaagggccggttcaccatctccagagacaattccaagaacacgctgtttctgcaaatgaacagcctgagagccgaggacacggccgtatattactgtgcgaaaatttttgggtcctactactttgactactggggccagggaaccctggtcacagtctcgagt

SEQ ID NO: 165 - DNA, 339 bp, synthetic construct
  misc_feature 1..339: note = source = /note="Description of Artificial Sequence: Synthetic polynucleotide"
  source 1..339: mol_type = other DNA
gaaattgtgatgacacagtctccagactccctggctgtgtctctgggcgagagggccaccatcaactgcaagtccagccagagtgttttatacagctccaacaataagaactacttagcttggtaccagcagaaaccaggacagcctcctaagctgctcatttactggacatctacccgggaatccggggtccctaaccgattcagtggcagcgggtctgggacagatttcactctcaccatcagcagcctgcaggctgaagatgtggcagtttattactgtcagcaatattatagtggtcctccgacgttcggccaagggaccaaggtggaaatcaaa

SEQ ID NO: 166 - protein, 118 aa, synthetic construct
  REGION 1..118: note = source = /note="Description of Artificial Sequence: Synthetic polypeptide"
QVQLQQSGGGLVQPGGSLRLSCAASGFTLSSYAMSWVRQAPGKGLEWVSGISGSGGSTYNADSVKGRFTISRDNSKNTLFLQMNSLRAEDTAVYYCAKIFGSYYFDYWGQGTLVTVSS

SEQ ID NO: 167 - protein, 113 aa, synthetic construct
  REGION 1..113: note = source = /note="Description of Artificial Sequence: Synthetic polypeptide"
EIVMTQSPDSLAVSLGERATINCKSSQSVLYSSNNKNYLAWYQQKPGQPPKLLIYWTSTRESGVPNRFSGSGSGTDFTLTISSLQAEDVAVYYCQQYYSGPPTFGQGTKVEIK

SEQ ID NO: 168 - protein, 8 aa, synthetic construct
  REGION 1..8: note = source = /note="Description of Artificial Sequence: Synthetic peptide"
GFTLSSYA

SEQ ID NO: 169 - protein, 8 aa, synthetic construct
  REGION 1..8: note = source = /note="Description of Artificial Sequence: Synthetic peptide"
ISGSGGST

SEQ ID NO: 170 - protein, 13 aa, synthetic construct
  REGION 1..13: note = source = /note="Description of Artificial Sequence: Synthetic peptide"
CAKIFGSYYFDYW

SEQ ID NO: 171 - protein, 12 aa, synthetic construct
  REGION 1..12: note = source = /note="Description of Artificial Sequence: Synthetic peptide"
QSVLYSSNNKNY

SEQ ID NO: 172 - skipped

SEQ ID NO: 173 - protein, 11 aa, synthetic construct [sequence omitted]

SEQ ID NO: 174 - DNA, 354 bp, synthetic construct
  misc_feature 1..354: note = source = /note="Description of Artificial Sequence: Synthetic polynucleotide"
  source 1..354: mol_type = other DNA
caggtgcagctggtggagtctgggggaggcttggttcggcctggggggtccctgagactctcctgtgcagtctctggattcacctttagcagctatgccatgagctgggtccgccaggctccagggaaggggctggagtgggtctcaggtattagtggtagtggtggtagcacatacaacgcagactccgtgaagggccggttcaccatctccagagacaattccaagaacacgctgtatcttcaaatgaacagcctgagagccgaggacacggccgtatattactgtgcgaaaatttttgggtcctactactttgactactggggccagggaaccctggtcaccgtctcgagt

SEQ ID NO: 175 - DNA, 339 bp, synthetic construct
  misc_feature 1..339: note = source = /note="Description of Artificial Sequence: Synthetic polynucleotide"
  source 1..339: mol_type = other DNA
gaaattgtgatgacacagtctccagactccctggctgtgtctctgggcgagagggccaccatcaactgcaagtccagccagagtgttttatacagctccaataataagaactacttagcttggtaccagcagaaatcaggacagcctcctaagctgctcatttactgggcatctacccgggaatccggggtccctgaccgattcagtggcagcgggtctgggacagatttcactctcaccatcagcagcctgcaggctgaagatgtggcagtttattactgtcagcaatattatagtggtccaccgacgttcggccaagggaccaaggtggaaatcaaa

SEQ ID NO: 176 - protein, 118 aa, synthetic construct
  REGION 1..118: note = source = /note="Description of Artificial Sequence: Synthetic polypeptide"
QVQLVESGGGLVRPGGSLRLSCAVSGFTFSSYAMSWVRQAPGKGLEWVSGISGSGGSTYNADSVKGRFTISRDNSKNTLYLQMNSLRAEDTAVYYCAKIFGSYYFDYWGQGTLVTVSS

SEQ ID NO: 177 - protein, 113 aa, synthetic construct
  REGION 1..113: note = source = /note="Description of Artificial Sequence: Synthetic polypeptide"
EIVMTQSPDSLAVSLGERATINCKSSQSVLYSSNNKNYLAWYQQKSGQPPKLLIYWASTRESGVPDRFSGSGSGTDFTLTISSLQAEDVAVYYCQQYYSGPPTFGQGTKVEIK

SEQ ID NO: 178 - protein, 8 aa, synthetic construct
  REGION 1..8: note = source = /note="Description of Artificial Sequence: Synthetic peptide"
GFTFSSYA

SEQ ID NO: 179 - protein, 8 aa, synthetic construct
  REGION 1..8: note = source = /note="Description of Artificial Sequence: Synthetic peptide"
ISGSGGST

SEQ ID NO: 180 - protein, 13 aa, synthetic construct
  REGION 1..13: note = source = /note="Description of Artificial Sequence: Synthetic peptide"
CAKIFGSYYFDYW

SEQ ID NO: 181 - protein, 12 aa, synthetic construct
  REGION 1..12: note = source = /note="Description of Artificial Sequence: Synthetic peptide"
QSVLYSSNNKNY

SEQ ID NO: 182 - skipped

SEQ ID NO: 183 - protein, 11 aa, synthetic construct [sequence omitted]

SEQ ID NO: 184 - DNA, 377 bp, synthetic construct
  misc_feature 1..377: note = source = /note="Description of Artificial Sequence: Synthetic polynucleotide"
  source 1..377: mol_type = other DNA
acgtgacagggcgcgcccaggtccagctgcaggagagcggtcccggactggtgaagccatcccagacactgagcctgacttgtactgtgagcggcggtagcatctccagcggcggctactattggtcctggatcaggcagcacccaggcaagggcctggagtggatcggctacatctactatagcggctctatctactataacccttccctgaagagccgggtgaccatctctgtggacacatccaagaatcagttctatctgaagctgtcttccgtgaccgccgctgatacagccgtgtactattgcgcctcactgatggtctggggggtcatgggcgattactgggggcagggcacactggtcacagtctcgagt

SEQ ID NO: 185 - DNA, 321 bp, synthetic construct
  misc_feature 1..321: note = source = /note="Description of Artificial Sequence: Synthetic polynucleotide"
  source 1..321: mol_type = other DNA
gagattgtgctgacccagtctcccgccaccctgtctctgagtcctggcgagagagccaccctgagctgcagagcctctcagtccgtgtccagctatctggcctggtatcagcagaagcccggccaggctccccggctgctgatctacgatgcctccaatagagccaccggcatccctgccagattctccggctctggctctggcaccgactttaccctgaccatctccagcctggaacccgaggacttcgccgtgtactactgccagcagcggtccgactggcctcctacatttggccaaggcaccaaggtggaaatcaag

SEQ ID NO: 186 - protein, 120 aa, synthetic construct
  REGION 1..120: note = source = /note="Description of Artificial Sequence: Synthetic polypeptide"
QVQLQESGPGLVKPSQTLSLTCTVSGGSISSGGYYWSWIRQHPGKGLEWIGYIYYSGSIYYNPSLKSRVTISVDTSKNQFYLKLSSVTAADTAVYYCASLMVWGVMGDYWGQGTLVTVSS

SEQ ID NO: 187 - protein, 107 aa, synthetic construct
  REGION 1..107: note = source = /note="Description of Artificial Sequence: Synthetic polypeptide"
EIVLTQSPATLSLSPGERATLSCRASQSVSSYLAWYQQKPGQAPRLLIYDASNRATGIPARFSGSGSGTDFTLTISSLEPEDFAVYYCQQRSDWPPTFGQGTKVEIK

SEQ ID NO: 188 - protein, 10 aa, synthetic construct
  REGION 1..10: note = source = /note="Description of Artificial Sequence: Synthetic peptide"
GGSISSGGYY

SEQ ID NO: 189 - protein, 7 aa, synthetic construct
  REGION 1..7: note = source = /note="Description of Artificial Sequence: Synthetic peptide"
IYYSGSI

SEQ ID NO: 190 - protein, 14 aa, synthetic construct
  REGION 1..14: note = source = /note="Description of Artificial Sequence: Synthetic peptide"
CASLMVWGVMGDYW

SEQ ID NO: 191 - protein, 6 aa, synthetic construct
  REGION 1..6: note = source = /note="Description of Artificial Sequence: Synthetic peptide"
QSVSSY

SEQ ID NO: 192 - skipped

SEQ ID NO: 193 - protein, 11 aa, synthetic construct [sequence omitted]

SEQ ID NO: 194 - DNA, 354 bp, synthetic construct
  misc_feature 1..354: note = source = /note="Description of Artificial Sequence: Synthetic polynucleotide"
  source 1..354: mol_type = other DNA
caggtccagctacagcagtctgggggaggcttggttcatcctggggggtccctaagactctcctgtgcagcctctggattcaccgttgacacctatgccatgacctgggtccgccaggctccagggaaggggctggagtgggtctcaggtattagcggtagtggtggtagcacatactacgcagactccgtgaagggccggttcaccatctccagagacaactccaagaacacgctgtatctgcaaatgaacagcctgagagacgaggacacggccgtatattactgtgcgaagatagtgggagttacccactttgactactggggccagggcaccctggtcacggtctcgagt

SEQ ID NO: 195 - DNA, 339 bp, synthetic construct
  misc_feature 1..339: note = source = /note="Description of Artificial Sequence: Synthetic polynucleotide"
  source 1..339: mol_type = other DNA
gaaattgtgatgacgcagtctccagactccctggctgtgtctctgggcgagagggccaccatcaactgcaagtccagccagagtgttttatacaggtccaacaataagaactatttagcttggtaccagcagaaaccaggacagcctcctaagctgctcatttactgggcatctacccgggaatccggggtccctgaccgattcagtggcagcgggtctgggacagatttcactctcaccatcagcagcctgcaggctgaagatgtggcagtttattactgtcagcaatattatagtggtccgatcaccttcggccaagggacacgactggagattaag

SEQ ID NO: 196 - protein, 118 aa, synthetic construct
  REGION 1..118: note = source = /note="Description of Artificial Sequence: Synthetic polypeptide"
QVQLQQSGGGLVHPGGSLRLSCAASGFTVDTYAMTWVRQAPGKGLEWVSGISGSGGSTYYADSVKGRFTISRDNSKNTLYLQMNSLRDEDTAVYYCAKIVGVTHFDYWGQGTLVTVSS

SEQ ID NO: 197 - protein, 113 aa, synthetic construct
  REGION 1..113: note = source = /note="Description of Artificial Sequence: Synthetic polypeptide"
EIVMTQSPDSLAVSLGERATINCKSSQSVLYRSNNKNYLAWYQQKPGQPPKLLIYWASTRESGVPDRFSGSGSGTDFTLTISSLQAEDVAVYYCQQYYSGPITFGQGTRLEIK

SEQ ID NO: 198 - protein, 8 aa, synthetic construct
  REGION 1..8: note = source = /note="Description of Artificial Sequence: Synthetic peptide"
GFTVDTYA

SEQ ID NO: 199 - protein, 8 aa, synthetic construct
  REGION 1..8: note = source = /note="Description of Artificial Sequence: Synthetic peptide"
ISGSGGST

SEQ ID NO: 200 - protein, 13 aa, synthetic construct
  REGION 1..13: note = source = /note="Description of Artificial Sequence: Synthetic peptide"
CAKIVGVTHFDYW

SEQ ID NO: 201 - protein, 12 aa, synthetic construct
  REGION 1..12: note = source = /note="Description of Artificial Sequence: Synthetic peptide"
QSVLYRSNNKNY

SEQ ID NO: 202 - skipped

SEQ ID NO: 203 - protein, 11 aa, synthetic construct [sequence omitted]

SEQ ID NO: 204 - DNA, 369 bp, synthetic construct
  misc_feature 1..369: note = source = /note="Description of Artificial Sequence: Synthetic polynucleotide"
  source 1..369: mol_type = other DNA
caggtcaccttgaaggagtcgggcccaggactggtgaagccttcacagaccctgtccctcacctgcactgtctctggtggctccatcagcagtggtggtcattactggagctggatccgccagcacccagggaagggcctggagtggattgggtacatctcttacagtgggagcacctactacaacccgtccctcaagagtcgacttaccatatcagtagacacgtctaagaaccagttctccctgaagctgagctctgtgactgccgcggacacggccgtgtattactgtgcgaccgcgtattacgatattttgactggttacccttttgactactggggccagggaaccctggtcacggtctcgagt

SEQ ID NO: 205 - DNA, 321 bp, synthetic construct
  misc_feature 1..321: note = source = /note="Description of Artificial Sequence: Synthetic polynucleotide"
  source 1..321: mol_type = other DNA
gaaattgtgatgacacagtctccagccaccctgtctttgtctccaggggaaagagccaccctctcctgcagggccagtcagagtgttagcagctacttagcctggtaccaacagaaacctggccaggctcccaggctcctcatctatgatgcatccgacagggccactggcatcccagccaggttcagtggcagtgggtctgggacagacttcactctcaccatcagcagcctagagcctgaagattttgcagtttattactgtcagcagcgtagcaactggccgatcaccttcggccaagggacacgactggagatcaag

SEQ ID NO: 206 - protein, 123 aa, synthetic construct
  REGION 1..123: note = source = /note="Description of Artificial Sequence: Synthetic polypeptide"
QVTLKESGPGLVKPSQTLSLTCTVSGGSISSGGHYWSWIRQHPGKGLEWIGYISYSGSTYYNPSLKSRLTISVDTSKNQFSLKLSSVTAADTAVYYCATAYYDILTGYPFDYWGQGTLVTVSS

SEQ ID NO: 207 - protein, 107 aa, synthetic construct
  REGION 1..107: note = source = /note="Description of Artificial Sequence: Synthetic polypeptide"
EIVMTQSPATLSLSPGERATLSCRASQSVSSYLAWYQQKPGQAPRLLIYDASDRATGIPARFSGSGSGTDFTLTISSLEPEDFAVYYCQQRSNWPITFGQGTRLEIK

SEQ ID NO: 208 - protein, 10 aa, synthetic construct
  REGION 1..10: note = source = /note="Description of Artificial Sequence: Synthetic peptide"
GGSISSGGHY

SEQ ID NO: 209 - protein, 7 aa, synthetic construct
  REGION 1..7: note = source = /note="Description of Artificial Sequence: Synthetic peptide"
ISYSGST

SEQ ID NO: 210 - protein, 17 aa, synthetic construct
  REGION 1..17: note = source = /note="Description of Artificial Sequence: Synthetic peptide"
CATAYYDILTGYPFDYW

SEQ ID NO: 211 - protein, 6 aa, synthetic construct
  REGION 1..6: note = source = /note="Description of Artificial Sequence: Synthetic peptide"
QSVSSY

SEQ ID NO: 212 - skipped

SEQ ID NO: 213 - protein, 11 aa, synthetic construct [sequence omitted]

SEQ ID NO: 214 - DNA, 369 bp, synthetic construct
  misc_feature 1..369: note = source = /note="Description of Artificial Sequence: Synthetic polynucleotide"
  source 1..369: mol_type = other DNA
caggtgcagctacagcagtcgggcccaggactggtgaagccttcacagaccctgtccctcacctgcactgtctctggtggctccatcagcagtggtggttactactggagctggatccgccagcacccagggaagggcctggagtggattgggtacatctcttatagtgggagtatctactacaacccgtccctcaagagtcgagttaccatatcagtagacacgtctaagaaccagttctccctgaagctgagctctgtgactgccacggacacggccgtgtattactgtgcgaccgcgtattacgatcttttgactggttacccttttgactactggggccagggaaccctggtcacggtctcgagt

SEQ ID NO: 215 - DNA, 321 bp, synthetic construct
  misc_feature 1..321: note = source = /note="Description of Artificial Sequence: Synthetic polynucleotide"
  source 1..321: mol_type = other DNA
gaaattgtgatgacgcagtctccagccaccctgtctttgtctccaggggaaagagccaccctctcctgcagggccagtcagagtgttagcagctacttagcctggtaccaacagaaacctggccaggctcccaggctcctcatctatgatgcatccaacagggccactggcatcccagccaggttcagtggcagtgggtctgggacagacttcactctcaccatcagcagcctagagcctgaagattttgcagtttattactgtcagcagcgtagcaactggccgatcaccttcggccaagggacacgactggagattaag

SEQ ID NO: 216 - protein, 123 aa, synthetic construct
  REGION 1..123: note = source = /note="Description of Artificial Sequence: Synthetic polypeptide"
QVQLQQSGPGLVKPSQTLSLTCTVSGGSISSGGYYWSWIRQHPGKGLEWIGYISYSGSIYYNPSLKSRVTISVDTSKNQFSLKLSSVTATDTAVYYCATAYYDLLTGYPFDYWGQGTLVTVSS

SEQ ID NO: 217 - protein, 107 aa, synthetic construct; identical to SEQ ID NO: 157
  REGION 1..107: note = source = /note="Description of Artificial Sequence: Synthetic polypeptide"

SEQ ID NO: 218 - protein, 10 aa, synthetic construct
  REGION 1..10: note = source = /note="Description of Artificial Sequence: Synthetic peptide"
GGSISSGGYY

SEQ ID NO: 219 - protein, 7 aa, synthetic construct
  REGION 1..7: note = source = /note="Description of Artificial Sequence: Synthetic peptide"
ISYSGSI

SEQ ID NO: 220 - protein, 17 aa, synthetic construct
  REGION 1..17: note = source = /note="Description of Artificial Sequence: Synthetic peptide"
CATAYYDLLTGYPFDYW

SEQ ID NO: 221 - protein, 6 aa, synthetic construct
  REGION 1..6: note = source = /note="Description of Artificial Sequence: Synthetic peptide"
QSVSSY

SEQ ID NO: 222 - skipped

SEQ ID NO: 223 - protein, 11 aa, synthetic construct [sequence omitted]

SEQ ID NO: 224 - DNA, 379 bp, synthetic construct
  misc_feature 1..379: note = source = /note="Description of Artificial Sequence: Synthetic polynucleotide"
  source 1..379: mol_type = other DNA
ggcgcgccgaggtgcagctgctggaatctggaggaggactggtccagccaggtggatccctgcgactgagctgcgccgcttctggattcacctttacaagatacgacatggtgtgggtccgccaggcaccaggaaagggactggagtgggtggctggtatcggcgatagtaacaagatgacccgctacgcacctgccgtcaaagggagggcaacaattagtcgggacaactcaaagaatactctgtatctgcagatgaattccctgcgagctgaggatacagcagtgtactattgtgccaaaggtagctgcatcgcctgttgggacgaagctggccgtattgatgcatggggacaggggactctggtgaccgtctcgag

SEQ ID NO: 225 - DNA, 351 bp, synthetic construct
  misc_feature 1..351: note = source = /note="Description of Artificial Sequence: Synthetic polynucleotide"
  source 1..351: mol_type = other DNA
gctagcctcttacgagctgactcaggaccctgcagtgagtgtcgccctgggccagacagtgagaatcacttgctccggcggagggagctacgatggttccagctactatggctggtatcagcagaagccaggacaggcacctgtgaccgtcatctataacaataacaataggccatctgacattcccgatcggttcagtggatctagttcagggaacacagcttctctgaccattacaggagcccaggctgaggacgaagcagattactattgtgggtcatacgacaggccagaaacaaattccgattatgtgggaatgtttggtagcggcactaaagtcaccgtcctagg

SEQ ID NO: 226 - protein, 124 aa, synthetic construct
  REGION 1..124: note = source = /note="Description of Artificial Sequence: Synthetic polypeptide"
EVQLLESGGGLVQPGGSLRLSCAASGFTFTRYDMVWVRQAPGKGLEWVAGIGDSNKMTRYAPAVKGRATISRDNSKNTLYLQMNSLRAEDTAVYYCAKGSCIACWDEAGRIDAWGQGTLVTVSS

SEQ ID NO: 227 - protein, 114 aa, synthetic construct
  REGION 1..114: note = source = /note="Description of Artificial Sequence: Synthetic polypeptide"
SYELTQDPAVSVALGQTVRITCSGGGSYDGSSYYGWYQQKPGQAPVTVIYNNNNRPSDIPDRFSGSSSGNTASLTITGAQAEDEADYYCGSYDRPETNSDYVGMFGSGTKVTVL

SEQ ID NO: 228 - protein, 8 aa, synthetic construct
  REGION 1..8: note = source = /note="Description of Artificial Sequence: Synthetic peptide"
GFTFTRYD

SEQ ID NO: 229 - protein, 8 aa, synthetic construct
  REGION 1..8: note = source = /note="Description of Artificial Sequence: Synthetic peptide"
IGDSNKMT

SEQ ID NO: 230 - protein, 19 aa, synthetic construct
  REGION 1..19: note = source = /note="Description of Artificial Sequence: Synthetic peptide"
CAKGSCIACWDEAGRIDAW

SEQ ID NO: 231 - protein, 8 aa, synthetic construct
  REGION 1..8: note = source = /note="Description of Artificial Sequence: Synthetic peptide"
GSYDGSSY

SEQ ID NO: 232 - skipped

SEQ ID NO: 233 - protein, 17 aa, synthetic construct
  REGION 1..17: note = source = /note="Description of Artificial Sequence: Synthetic peptide"
CGSYDRPETNSDYVGMF

SEQ ID NO: 234 - DNA, 400 bp, synthetic construct
  misc_feature 1..400: note = source = /note="Description of Artificial Sequence: Synthetic polynucleotide"
  source 1..400: mol_type = other DNA
ggcgcgccgaggtgcagctgctggaaagcggaggaggactggtccagccaggtggatctctgcgactgagttgcgccgcttcaggcttcacattttctgactacgccatgaactgggtgaggcaggctcctggcaagggactggagtgggtcgcaggaatcgggaacgatggaagttacactaattatggagcagccgtgaaggggagagctactatttcccgcgacaacagcaaaaataccctgtacctgcagatgaactcactgagagctgaagataccgcagtgtactattgtgcctctgacatcaggagtcggaatgattgctcctatttcctgggagggtgttccagcggctttattgacgtgtggggtcagggcaccctggtcacagtctcgag

SEQ ID NO: 235 - DNA, 321 bp, synthetic construct
  misc_feature 1..321: note = source = /note="Description of Artificial Sequence: Synthetic polynucleotide"
  source 1..321: mol_type = other DNA
gctagcctcttacgagctgacccaggacccagcagtgtccgtcgccctgggccagacagtgagaatcacttgctccggcggatccagctacagctatgggtggttccagcagaagcccggtcaggcccctgtgaccgtcatctatgaaagtaacaataggccatcagacattcccgatcggttttctggctctagttcaggaaacacagctagtctgaccatcacaggggcccaggctgaggacgaagctgattactattgtggcaatgcagattccagctctggaattttcgggtccggtactaaagtcaccgtcctagg

SEQ ID NO: 236 - protein, 131 aa, synthetic construct
  REGION 1..131: note = source = /note="Description of Artificial Sequence: Synthetic polypeptide"
EVQLLESGGGLVQPGGSLRLSCAASGFTFSDYAMNWVRQAPGKGLEWVAGIGNDGSYTNYGAAVKGRATISRDNSKNTLYLQMNSLRAEDTAVYYCASDIRSRNDCSYFLGGCSSGFIDVWGQGTLVTVSS

SEQ ID NO: 237 - protein, 104 aa, synthetic construct
  REGION 1..104: note = source = /note="Description of Artificial Sequence: Synthetic polypeptide"
SYELTQDPAVSVALGQTVRITCSGGSSYSYGWFQQKPGQAPVTVIYESNNRPSDIPDRFSGSSSGNTASLTITGAQAEDEADYYCGNADSSSGIFGSGTKVTVL

SEQ ID NO: 238 - protein, 8 aa, synthetic construct
  REGION 1..8: note = source = /note="Description of Artificial Sequence: Synthetic peptide"
GFTFSDYA

SEQ ID NO: 239 - protein, 8 aa, synthetic construct
  REGION 1..8: note = source = /note="Description of Artificial Sequence: Synthetic peptide"
IGNDGSYT

SEQ ID NO: 240 - protein, 26 aa, synthetic construct
  REGION 1..26: note = source = /note="Description of Artificial Sequence: Synthetic peptide"
CASDIRSRNDCSYFLGGCSSGFIDVW

SEQ ID NO: 241 - protein, 4 aa, synthetic construct
  REGION 1..4: note = source = /note="Description of Artificial Sequence: Synthetic peptide"
SSYS

SEQ ID NO: 242 - skipped

SEQ ID NO: 243 - protein, 11 aa, synthetic construct
  REGION 1..11: note = source = /note="Description of Artificial Sequence: Synthetic peptide"
CGNADSSSGIF

SEQ ID NO: 244 - DNA, 385 bp, synthetic construct
  misc_feature 1..385: note = source = /note="Description of Artificial Sequence: Synthetic polynucleotide"
  source 1..385: mol_type = other DNA
ggcgcgccgaggtgcagctgctggaatccggaggaggactggtccagccaggtggatccctgcgactgagctgcgccgcttctggattcgactttagcgatcacgggatgcagtgggtgagacaggcaccaggcaagggactggagtacgtgggtgtcatcgacaccacaggccgctatacatactatgcacctgccgtcaagggcagggctaccattagtcgggacaactcaaaaaatacactgtacctgcagatgaactctctgagggctgaagatactgcagtgtactattgcgccaaaactacctgcgtgggagggtacctgtgcaataccgtcggaagtatcgatgcttggggacaggggacactggtgactgtctcgag

SEQ ID NO: 245 - DNA, 330 bp, synthetic construct
  misc_feature 1..330: note = source = /note="Description of Artificial Sequence: Synthetic polynucleotide"
  source 1..330: mol_type = other DNA
gctagcctcctacgagctgactcaggacccagcagtgagcgtcgccctgggccagacagtgagaatcacttgctctggcggagggtccagctcttactatggttggtaccagcagaagcccggccaggctcctgtgaccgtcatctatgacgatacaaacaggccaagtggaattcccgatcggttctcaggtagttcatccggcaatacagcttctctgaccatcacaggggcccaggctgaggacgaagcagattactattgtggtggctatgaaggaagctctcacgccgggatttttggaagtgggactaaagtcaccgtcctagg

SEQ ID NO: 246 - protein, 126 aa, synthetic construct
  REGION 1..126: note = source = /note="Description of Artificial Sequence: Synthetic polypeptide"
EVQLLESGGGLVQPGGSLRLSCAASGFDFSDHGMQWVRQAPGKGLEYVGVIDTTGRYTYYAPAVKGRATISRDNSKNTLYLQMNSLRAEDTAVYYCAKTTCVGGYLCNTVGSIDAWGQGTLVTVSS

SEQ ID NO: 247 - protein, 107 aa, synthetic construct
  REGION 1..107: note = source = /note="Description of Artificial Sequence: Synthetic polypeptide"
SYELTQDPAVSVALGQTVRITCSGGGSSSYYGWYQQKPGQAPVTVIYDDTNRPSGIPDRFSGSSSGNTASLTITGAQAEDEADYYCGGYEGSSHAGIFGSGTKVTVL

SEQ ID NO: 248 - protein, 8 aa, synthetic construct
  REGION 1..8: note = source = /note="Description of Artificial Sequence: Synthetic peptide"
GFDFSDHG

SEQ ID NO: 249 - protein, 8 aa, synthetic construct
  REGION 1..8: note = source = /note="Description of Artificial Sequence: Synthetic peptide"
IDTTGRYT

SEQ ID NO: 250 - protein, 21 aa, synthetic construct
  REGION 1..21: note = source = /note="Description of Artificial Sequence: Synthetic peptide"
CAKTTCVGGYLCNTVGSIDAW

SEQ ID NO: 251 - protein, 5 aa, synthetic construct
  REGION 1..5: note = source = /note="Description of Artificial Sequence: Synthetic peptide"
GSSSY

SEQ ID NO: 252 - skipped

SEQ ID NO: 253 - protein, 13 aa, synthetic construct
  REGION 1..13: note = source = /note="Description of Artificial Sequence: Synthetic peptide"
CGGYEGSSHAGIF

SEQ ID NO: 254 - DNA, 376 bp, synthetic construct
  misc_feature 1..376: note = source = /note="Description of Artificial Sequence: Synthetic polynucleotide"
  source 1..376: mol_type = other DNA
ggcgcgccgaggtgcagctgctggaaagtggaggaggactggtccagccaggtggaagcctgagactgtcttgcgccgctagtggcttcgacttttccagctacaccatgcagtgggtgaggcaggcaccaggcaagggactggagtgggtgggcgtcatctctagtactggagggtctaccggatacgggcctgctgtgaagggaagggcaacaatttcacgggataactccaaaaatactctgtatctgcagatgaacagcctgagggcagaagacacagccgtgtactattgcgtgaaatcaatctccggagatgcctggtctgtggacgggctggatgcttggggtcagggcaccctggtcacagtctcgag

SEQ ID NO: 255 - DNA, 321 bp, synthetic construct
  misc_feature 1..321: note = source = /note="Description of Artificial Sequence: Synthetic polynucleotide"
  source 1..321: mol_type = other DNA
gctagcctcatacgagctgacccaggacccagcagtgtccgtcgccctgggacagacagtgagaatcacttgctccggaggaggatccgcctacggttggtatcagcagaagcccggccaggcacctgtgaccgtcatctactataacaatcagaggccatctggcattcccgaccggttcagtggatccagctctgggaacacagcaagtctgaccatcacaggcgcccaggctgaggacgaagccgattactattgtggaagctatgatagttcagctgtggggatttttggttctggcactaaagtcaccgtcctagg

SEQ ID NO: 256 - protein, 123 aa, synthetic construct
  REGION 1..123: note = source = /note="Description of Artificial Sequence: Synthetic polypeptide"
EVQLLESGGGLVQPGGSLRLSCAASGFDFSSYTMQWVRQAPGKGLEWVGVISSTGGSTGYGPAVKGRATISRDNSKNTLYLQMNSLRAEDTAVYYCVKSISGDAWSVDGLDAWGQGTLVTVSS

SEQ ID NO: 257 - protein, 104 aa, synthetic construct
  REGION 1..104: note = source = /note="Description of Artificial Sequence: Synthetic polypeptide"
SYELTQDPAVSVALGQTVRITCSGGGSAYGWYQQKPGQAPVTVIYYNNQRPSGIPDRFSGSSSGNTASLTITGAQAEDEADYYCGSYDSSAVGIFGSGTKVTVL

SEQ ID NO: 258 - protein, 8 aa, synthetic construct
  REGION 1..8: note = source = /note="Description of Artificial Sequence: Synthetic peptide"
GFDFSSYT

SEQ ID NO: 259 - protein, 8 aa, synthetic construct
  REGION 1..8: note = source = /note="Description of Artificial Sequence: Synthetic peptide"
ISSTGGST

SEQ ID NO: 260 - protein, 18 aa, synthetic construct
  REGION 1..18: note = source = /note="Description of Artificial Sequence: Synthetic peptide"
CVKSISGDAWSVDGLDAW

SEQ ID NO: 261-262 - skipped (2 entries)

SEQ ID NO: 263 - protein, 12 aa, synthetic construct
  REGION 1..12: note = source = /note="Description of Artificial Sequence: Synthetic peptide"
CGSYDSSAVGIF

SEQ ID NO: 264 - DNA, 376 bp, synthetic construct
  misc_feature 1..376: note = source = /note="Description of Artificial Sequence: Synthetic polynucleotide"
  source 1..376: mol_type = other DNA
ggcgcgccgaggtgcagctgctggaaagtggaggaggactggtccagccaggtggaagcctgagactgtcttgcgccgctagtggcttcgacttttccagctacaccatgcagtgggtgaggcaggcaccaggcaagggactggagtgggtgggcgtcatctctagtactggagggtctaccggatacgggcctgctgtgaagggaagggcaacaatttcacgggataactccaaaaatactctgtatctgcagatgaacagcctgagggcagaagacacagccgtgtactattgcgtgaaatcagtctccggagatgcctggtctgtggacgggctggatgcttggggtcagggcaccctggtcacagtctcgag

SEQ ID NO: 265 - DNA, 321 bp, synthetic construct
  misc_feature 1..321: note = source = /note="Description of Artificial Sequence: Synthetic polynucleotide"
  source 1..321: mol_type = other DNA
gctagcctcatacgagctgacccaggacccagcagtgtccgtcgccctgggccagacagtgagaatcacttgctccggaggaggatccgcctacggttggtatcagcagaagcccggccaggcacctgtgaccgtcatctactataacaatcagaggccatctgacattcccgatcggttcagtggatccagctctgggaacacagcaagtctgaccatcacaggcgcccaggctgaggacgaagccgattactattgtggaagctatgatagttcagctgtggggatttttggttctggcactaaagtcaccgtcctagg

SEQ ID NO: 266 - protein, 123 aa, synthetic construct
  REGION 1..123: note = source = /note="Description of Artificial Sequence: Synthetic polypeptide"
EVQLLESGGGLVQPGGSLRLSCAASGFDFSSYTMQWVRQAPGKGLEWVGVISSTGGSTGYGPAVKGRATISRDNSKNTLYLQMNSLRAEDTAVYYCVKSVSGDAWSVDGLDAWGQGTLVTVSS

SEQ ID NO: 267 - protein, 104 aa, synthetic construct
  REGION 1..104: note = source = /note="Description of Artificial Sequence: Synthetic polypeptide"
SYELTQDPAVSVALGQTVRITCSGGGSAYGWYQQKPGQAPVTVIYYNNQRPSDIPDRFSGSSSGNTASLTITGAQAEDEADYYCGSYDSSAVGIFGSGTKVTVL

SEQ ID NO: 268 - protein, 8 aa, synthetic construct
  REGION 1..8: note = source = /note="Description of Artificial Sequence: Synthetic peptide"
GFDFSSYT

SEQ ID NO: 269 - protein, 8 aa, synthetic construct
  REGION 1..8: note = source = /note="Description of Artificial Sequence: Synthetic peptide"
ISSTGGST

SEQ ID NO: 270 - protein, 18 aa, synthetic construct
  REGION 1..18: note = source = /note="Description of Artificial Sequence: Synthetic peptide"
CVKSVSGDAWSVDGLDAW

SEQ ID NO: 271-272 - skipped (2 entries)

SEQ ID NO: 273 - protein, 12 aa, synthetic construct
  REGION 1..12: note = source = /note="Description of Artificial Sequence: Synthetic peptide"
CGSYDSSAVGIF

SEQ ID NO: 274 - DNA, 385 bp, synthetic construct
  misc_feature 1..385: note = source = /note="Description of Artificial Sequence: Synthetic polynucleotide"
  source 1..385: mol_type = other DNA
ggcgcgccgaggtgcagctgctggaatccggaggaggactggtccagccaggtggaagcctgcgactgtcttgcgccgctagtggattcgacttttccagctacggaatgcagtgggtgaggcaggcaccaggcaagggactggagtgggtgggcgtcatctctggaagtgggattaccacactgtacgcacctgccgtcaagggaagggctactatctcacgggacaactctaaaaatacagtgtatctgcagatgaactccctgagagctgaagataccgcagtctactattgtacacgctcaccctccatcacagacggctggacttatggaggggcctggattgatgcttggggtcagggcactctggtgaccgtctcgag

SEQ ID NO: 275 - DNA, 318 bp, synthetic construct
  misc_feature 1..318: note = source = /note="Description of Artificial Sequence: Synthetic polynucleotide"
  source 1..318: mol_type = other DNA
gctagccagctacgagctgacccaggacccagcagtgtccgtcgccctgggccagacagtgagaatcacttgcagtggcggagatgggtcatacggttggttccagcagaagcccggacaggcccctgtgaccgtcatctatgacaacgataataggccatctgacattcccgatcggtttagtggctccagctctggaaacacagcttctctgaccatcacaggggcccaggctgaggacgaagctgattactattgtggcaatgcagacctgtccgggggtattttcggcagcggaactaaagtcaccgtcctagg

SEQ ID NO: 276 - protein, 126 aa, synthetic construct
  REGION 1..126: note = source = /note="Description of Artificial Sequence: Synthetic polypeptide"
EVQLLESGGGLVQPGGSLRLSCAASGFDFSSYGMQWVRQAPGKGLEWVGVISGSGITTLYAPAVKGRATISRDNSKNTVYLQMNSLRAEDTAVYYCTRSPSITDGWTYGGAWIDAWGQGTLVTVSS

SEQ ID NO: 277 - protein, 103 aa, synthetic construct
  REGION 1..103: note = source = /note="Description of Artificial Sequence: Synthetic polypeptide"
SYELTQDPAVSVALGQTVRITCSGGDGSYGWFQQKPGQAPVTVIYDNDNRPSDIPDRFSGSSSGNTASLTITGAQAEDEADYYCGNADLSGGIFGSGTKVTVL

SEQ ID NO: 278 - protein, 8 aa, synthetic construct
  REGION 1..8: note = source = /note="Description of Artificial Sequence: Synthetic peptide"
GFDFSSYG

SEQ ID NO: 279 - protein, 8 aa, synthetic construct
  REGION 1..8: note = source = /note="Description of Artificial Sequence: Synthetic peptide"
ISGSGITT

SEQ ID NO: 280 - protein, 21 aa, synthetic construct
  REGION 1..21: note = source = /note="Description of Artificial Sequence: Synthetic peptide"
CTRSPSITDGWTYGGAWIDAW

SEQ ID NO: 281-282 - skipped (2 entries)

SEQ ID NO: 283 - protein, 11 aa, synthetic construct
  REGION 1..11: note = source = /note="Description of Artificial Sequence: Synthetic peptide"
CGNADLSGGIF

SEQ ID NO: 284 - DNA, 388 bp, synthetic construct
  misc_feature 1..388: note = source = /note="Description of Artificial Sequence: Synthetic polynucleotide"
  source 1..388: mol_type = other DNA
ggcgcgccgaggtgcagctgctggaatctggaggaggactggtccagccaggtggatccctgagactgagctgcgccgcttctggattcacctttagtacattcaacatggtgtgggtcaggcaggcacctggaaagggactggagtacgtggctgaaatctccagcgacggctcttttacatggtatgcaactgccgtcaagggcagggccaccattagtcgggataactcaaaaaatacagtgtacctgcagatgaattccctgagggctgaggacaccgcagtctactattgcgcaaaatccgattgttctagttcatactatggatatagctgtatcgggatcattgacgcttggggtcagggcactctggtgaccgtctcgag

SEQ ID NO: 285 - DNA, 339 bp, synthetic construct
  misc_feature 1..339: note = source = /note="Description of Artificial Sequence: Synthetic polynucleotide"
  source 1..339: mol_type = other DNA
gctagcctcctatgagctgacccaggacccagcagtgagcgtcgccctgggccagacagtgagaatcacttgctccggcggaattagcgacgatggctcttactattacggatggttccagcagaagcccggacaggcccctgtgaccgtcatctatattaacgacaggcggccaagtaatatccccgataggttttcagggtccagctctggtaacacagcttctctgaccattacaggggcccaggctgaggacgaagctgattattactgtggctcttacgatagttcagcaggggtgggtatcttcggcagtggaactaaagtcaccgtcctagg

SEQ ID NO: 286 - protein, 127 aa, synthetic construct
  REGION 1..127: note = source = /note="Description of Artificial Sequence: Synthetic polypeptide"
EVQLLESGGGLVQPGGSLRLSCAASGFTFSTFNMVWVRQAPGKGLEYVAEISSDGSFTWYATAVKGRATISRDNSKNTVYLQMNSLRAEDTAVYYCAKSDCSSSYYGYSCIGIIDAWGQGTLVTVSS

SEQ ID NO: 287 - protein, 110 aa, synthetic construct
  REGION 1..110: note = source = /note="Description of Artificial Sequence: Synthetic polypeptide"
SYELTQDPAVSVALGQTVRITCSGGISDDGSYYYGWFQQKPGQAPVTVIYINDRRPSNIPDRFSGSSSGNTASLTITGAQAEDEADYYCGSYDSSAGVGIFGSGTKVTVL

SEQ ID NO: 288 - protein, 8 aa, synthetic construct
  REGION 1..8: note = source = /note="Description of Artificial Sequence: Synthetic peptide"
GFTFSTFN

SEQ ID NO: 289 - protein, 8 aa, synthetic construct
  REGION 1..8: note = source = /note="Description of Artificial Sequence: Synthetic peptide"
ISSDGSFT

SEQ ID NO: 290 - protein, 22 aa, synthetic construct
  REGION 1..22: note = source = /note="Description of Artificial Sequence: Synthetic peptide"
CAKSDCSSSYYGYSCIGIIDAW

SEQ ID NO: 291 - protein, 8 aa, synthetic construct
  REGION 1..8: note = source = /note="Description of Artificial Sequence: Synthetic peptide"
ISDDGSYY

SEQ ID NO: 292 - skipped

SEQ ID NO: 293 - protein, 13 aa, synthetic construct
  REGION 1..13: note = source = /note="Description of Artificial Sequence: Synthetic peptide"
CGSYDSSAGVGIF

SEQ ID NO: 294 - DNA, 400 bp, synthetic construct
  misc_feature 1..400: note = source = /note="Description of Artificial Sequence: Synthetic polynucleotide"
  source 1..400: mol_type = other DNA
ggcgcgccgaggtgcagctgctggaaagtggaggaggactggtccagccaggtggatcactgagactgtcctgcgccgcctccggcttcaccttttccagctacaacatgttctgggtgcgccaggcaccaggaaagggactggagtttgtcgctgaaatctctggtagtaatactggaagccgaacctggtacgcacctgccgtgaagggcagggctacaatttctcgggacaacagtaaaaatactctgtatctgcagatgaactctctgagggctgaggatacagcagtgtactattgtgcaaaatcaatctacggagggtattgcgccggtggctattcctgtggtgtgggcctgattgacgcatggggacaggggaccctggtcacagtctcgag

SEQ ID NO: 295 - DNA, 321 bp, synthetic construct
  misc_feature 1..321: note = source = /note="Description of Artificial Sequence: Synthetic polynucleotide"
  source 1..321: mol_type = other DNA
gctagcctcatacgagctgacccaggacccagcagtgtccgtcgccctgggccagacagtgagaatcacttgcagtggcggatccagcgattactatgggtggttccagcagaagcccggtcaggcccctgtgaccgtcatctactataacaacaagaggccatctgacattcccgatcggtttagtggctctagttcaggaaacacagcctccctgaccattacaggggcccaggctgaggacgaagctgattactattgtggcaatgcagactccagcgtgggagtcttcgggtctggtactaaggtgaccgtcctagg

SEQ ID NO: 296 - protein, 131 aa, synthetic construct
  REGION 1..131: note = source = /note="Description of Artificial Sequence: Synthetic polypeptide"
EVQLLESGGGLVQPGGSLRLSCAASGFTFSSYNMFWVRQAPGKGLEFVAEISGSNTGSRTWYAPAVKGRATISRDNSKNTLYLQMNSLRAEDTAVYYCAKSIYGGYCAGGYSCGVGLIDAWGQGTLVTVSS

SEQ ID NO: 297 - protein, 104 aa, synthetic construct
  REGION 1..104: note = source = /note="Description of Artificial Sequence: Synthetic polypeptide"
SYELTQDPAVSVALGQTVRITCSGGSSDYYGWFQQKPGQAPVTVIYYNNKRPSDIPDRFSGSSSGNTASLTITGAQAEDEADYYCGNADSSVGVFGSGTKVTVL

SEQ ID NO: 298 - protein, 8 aa, synthetic construct
  REGION 1..8: note = source = /note="Description of Artificial Sequence: Synthetic peptide"
GFTFSSYN

SEQ ID NO: 299 - protein, 10 aa, synthetic construct
  REGION 1..10: note = source = /note="Description of Artificial Sequence: Synthetic peptide"
ISGSNTGSRT

SEQ ID NO: 300 - protein, 24 aa, synthetic construct
  REGION 1..24: note = source = /note="Description of Artificial Sequence: Synthetic peptide"
CAKSIYGGYCAGGYSCGVGLIDAW

SEQ ID NO: 301 - protein, 4 aa, synthetic construct
  REGION 1..4: note = source = /note="Description of Artificial Sequence: Synthetic peptide"
SSDY

SEQ ID NO: 302 - skipped

SEQ ID NO: 303 - protein, 11 aa, synthetic construct
  REGION 1..11: note = source = /note="Description of Artificial Sequence: Synthetic peptide"
CGNADSSVGVF

SEQ ID NO: 304 - DNA, 357 bp, synthetic construct
  misc_feature 1..357: note = source = /note="Description of Artificial Sequence: Synthetic polynucleotide"
  source 1..357: mol_type = other DNA
caggtgcagctgcagcagtggggtgccggtctgctgaagccttctgaaactctgtctctgacttgtgccgtctatggtggatcattcagcggctactattggtcctggatcaggcagccccctggcaagggcctggagtggatcggcgagatcaaccaccggggctctaccaactacaatccctctctgaagagcagggtgaccatctccgtggacacatctaagaatcagttcagcctgaagctgagctccgtgaccgccgctgatacagccgtgtactattgcacaaggggggaggaatgggagtcactgttctttgattactgggggcaggggacactggtcacagtctcgagt

SEQ ID NO: 305 - DNA, 321 bp, synthetic construct
  misc_feature 1..321: note = source = /note="Description of Artificial Sequence: Synthetic polynucleotide"
  source 1..321: mol_type = other DNA
gaaatcgtcctgacccagtcccccgccaccctgagcctgagccccggagaaagagccaccctgtcctgccgagcaagccagtccatcagctcctatctcgcctggtatcagcagaaaccaggccaggctccccggctgctgatctacggcgcctccaacagagctacaggaatcccagcccgcttcagcggctccggctctggcacagactttaccctgacaatctctagcctggagcctgaggatttcgccgtgtactattgccagcagagatctaattggccactgacattcggcggcggcacacgggtggagatcaag

SEQ ID NO: 306 - protein, 119 aa, synthetic construct
  REGION 1..119: note = source = /note="Description of Artificial Sequence: Synthetic polypeptide"
QVQLQQWGAGLLKPSETLSLTCAVYGGSFSGYYWSWIRQPPGKGLEWIGEINHRGSTNYNPSLKSRVTISVDTSKNQFSLKLSSVTAADTAVYYCTRGEEWESLFFDYWGQGTLVTVSS

SEQ ID NO: 307 - protein, 107 aa, synthetic construct
  REGION 1..107: note = source = /note="Description of Artificial Sequence: Synthetic polypeptide"
EIVLTQSPATLSLSPGERATLSCRASQSISSYLAWYQQKPGQAPRLLIYGASNRATGIPARFSGSGSGTDFTLTISSLEPEDFAVYYCQQRSNWPLTFGGGTRVEIK

SEQ ID NO: 308 - protein, 8 aa, synthetic construct
  REGION 1..8: note = source = /note="Description of Artificial Sequence: Synthetic peptide"
GGSFSGYY

SEQ ID NO: 309 - protein, 7 aa, synthetic construct
  REGION 1..7: note = source = /note="Description of Artificial Sequence: Synthetic peptide"
INHRGST

SEQ ID NO: 310 - protein, 15 aa, synthetic construct
  REGION 1..15: note = source = /note="Description of Artificial Sequence: Synthetic peptide"
CTRGEEWESLFFDYW

SEQ ID NO: 311 - protein, 6 aa, synthetic construct
  REGION 1..6: note = source = /note="Description of Artificial Sequence: Synthetic peptide"
QSISSY

SEQ ID NO: 312 - skipped

SEQ ID NO: 313 - protein, 11 aa, synthetic construct [sequence omitted]

SEQ ID NO: 314 - DNA, 366 bp, synthetic construct
  misc_feature 1..366: note = source = /note="Description of Artificial Sequence: Synthetic polynucleotide"
  source 1..366: mol_type = other DNA
caggttcagctgcagcagtggggcgccggcctgctgagaccaagcgagaccctgtccctgacatgcgccgtgtatggcgagagcttctccggctattactggaactggatccggcagcctcccggcaagggcctggagtggatcggcgagatcaatcactccggctccaccaattacaacccatccctgaagtctcgggtgacaatcagcgtggatacaagcaagacccagttcagcctgaagctgagctccgtgacagctgccgataccgccgtgtattactgcgccagaggctgggacctgctggattggaatgactactggaatgagtactggggccaggggaccctggtgaccgtctcgagt

SEQ ID NO: 315 - DNA, 321 bp, synthetic construct
  misc_feature 1..321: note = source = /note="Description of Artificial Sequence: Synthetic polynucleotide"
  source 1..321: mol_type = other DNA
gagatcgtgctgacccagtcccctgccaccctgtctctgtcccctggcgagcgggccaccctgtcctgtagagcttctcagtccgtgtcttcctacctggcttggtaccagcagaagccaggacaggccccaagactgctgatctatgacgcttccaatcgggctaccggcatcccagctcgctttagcggctccggctccggcaccgacttcaccctgacaatcagctccctggagccagaggattttgccgtgtattactgtcagcagaggtccaattggccactgacatttggcggcggcacaaaggttgagatcaag

SEQ ID NO: 316 - protein, 122 aa, synthetic construct
  REGION 1..122: note = source = /note="Description of Artificial Sequence: Synthetic polypeptide"
QVQLQQWGAGLLRPSETLSLTCAVYGESFSGYYWNWIRQPPGKGLEWIGEINHSGSTNYNPSLKSRVTISVDTSKTQFSLKLSSVTAADTAVYYCARGWDLLDWNDYWNEYWGQGTLVTVSS

SEQ ID NO: 317 - protein, 107 aa, synthetic construct; identical to SEQ ID NO: 4
  REGION 1..107: note = source = /note="Description of Artificial Sequence: Synthetic polypeptide"

SEQ ID NO: 318 - protein, 8 aa, synthetic construct
  REGION 1..8: note = source = /note="Description of Artificial Sequence: Synthetic peptide"
GESFSGYY

SEQ ID NO: 319 - protein, 7 aa, synthetic construct
  REGION 1..7: note = source = /note="Description of Artificial Sequence: Synthetic peptide"
INHSGST

SEQ ID NO: 320 - protein, 18 aa, synthetic construct
  REGION 1..18: note = source = /note="Description of Artificial Sequence: Synthetic peptide"
CARGWDLLDWNDYWNEYW

SEQ ID NO: 321 - protein, 6 aa, synthetic construct
  REGION 1..6: note = source = /note="Description of Artificial Sequence: Synthetic peptide"
QSVSSY

SEQ ID NO: 322 - skipped

SEQ ID NO: 323 - protein, 11 aa, synthetic construct [sequence omitted]

SEQ ID NO: 324 - DNA, 357 bp, synthetic construct
  misc_feature 1..357: note = source = /note="Description of Artificial Sequence: Synthetic polynucleotide"
  source 1..357: mol_type = other DNA
caggttcagctgcagcagtggggcgctggcctgctgaagccctctgagaccctgtctctgacctgtgccgtgtatggcggcagcttctccggctattactggaactggatccgccagccccccggcaagggcctggagtggatcggcgagatcaaccactccggctctaccaactacaatccttctctgaagtccagggtgacaatcagcgtggacaccagcaagaaccagtttagcctgaagctgtccagcgtgacagctgccgatacagccgtgtattactgcgccagaggcgaggattggggcgagagcttctttgattactggggccaggggaccctggtgaccgtctcgagt

SEQ ID NO: 325 - DNA, 321 bp, synthetic construct
  misc_feature 1..321: note = source = /note="Description of Artificial Sequence: Synthetic polynucleotide"
  source 1..321: mol_type = other DNA
gagatcgtgctgacccagtcccctgccaccctgtctctgtcccctggcgagcgggccaccctgagctgtcgggcctcccagtccgtgagctcctacctggcttggtatcagcagaagccaggacaggccccaagactgctgatctacgccgcttccaatcgggccaccggcatccccgccagattttccggctctggctccggcaccgatttcaccctgacaatcagctccctggagccagaggacttcgccgtgtactactgccagcagaggtctaattggccactgacatttggcggcggcaccaaggttgagatcaag

SEQ ID NO: 326 - protein, 119 aa, synthetic construct
  REGION 1..119: note = source = /note="Description of Artificial Sequence: Synthetic polypeptide"
QVQLQQWGAGLLKPSETLSLTCAVYGGSFSGYYWNWIRQPPGKGLEWIGEINHSGSTNYNPSLKSRVTISVDTSKNQFSLKLSSVTAADTAVYYCARGEDWGESFFDYWGQGTLVTVSS

SEQ ID NO: 327 - protein, 107 aa, synthetic construct
  REGION 1..107: note = source = /note="Description of Artificial Sequence: Synthetic polypeptide"
EIVLTQSPATLSLSPGERATLSCRASQSVSSYLAWYQQKPGQAPRLLIYAASNRATGIPARFSGSGSGTDFTLTISSLEPEDFAVYYCQQRSNWPLTFGGGTKVEIK

SEQ ID NO: 328 - protein, 8 aa, synthetic construct
  REGION 1..8: note = source = /note="Description of Artificial Sequence: Synthetic peptide"
GGSFSGYY

SEQ ID NO: 329 - protein, 7 aa, synthetic construct
  REGION 1..7: note = source = /note="Description of Artificial Sequence: Synthetic peptide"
INHSGST

SEQ ID NO: 330 - protein, 15 aa, synthetic construct
  REGION 1..15: note = source = /note="Description of Artificial Sequence: Synthetic peptide"
CARGEDWGESFFDYW

SEQ ID NO: 331 - protein, 6 aa, synthetic construct
  REGION 1..6: note = source = /note="Description of Artificial Sequence: Synthetic peptide"
QSVSSY

SEQ ID NO: 332 - skipped

SEQ ID NO: 333 - protein, 11 aa, synthetic construct [sequence omitted]

SEQ ID NO: 334 - DNA, 357 bp, synthetic construct
  misc_feature 1..357: note = source = /note="Description of Artificial Sequence: Synthetic polynucleotide"
  source 1..357: mol_type = other DNA
caggttcagctggtgcagtccggcgctgaggtgaagaagcctggagcttctgtgaaggtttcctgtaaggtttccggctatagcctgaccgagatctctatgcactgggtacggcaagcccccggcaagggcctggagtggatgggcggctttgacccagaggatggcgagaccatctacgctcagaggtttcaggggcgcgtgatcatgaccgaggataccagcaccgataccgcctacatggagctgtccagcctgagatccgaggataccgccgtgtattactgcgctactggtggctggggccccaattggttcgatccttggggccaggggaccctggtgaccgtctcgagt

SEQ ID NO: 335 - DNA, 321 bp, synthetic construct
  misc_feature 1..321: note = source = /note="Description of Artificial Sequence: Synthetic polynucleotide"
  source 1..321: mol_type = other DNA
gacatccagatgacacagtctccttcctctgtgagcgcctctgtgggcgaccgcgtgaccatcacatgccgcgcttcccaggggatctcttcctggctggcttggtaccagcagaagcccggcaaggcccccaagctgctgatctatgctgccagcagcctgcagtccggcgtgccttccaggtttagcggctccggctccggcaccgactttacactgacaatcagctccctgcagcccgaggattttgccacctattactgtcagcaggcgaattccttcccttttacattcggccctggcaccaaggttgatatcaag

SEQ ID NO: 336 - protein, 119 aa, synthetic construct
  REGION 1..119: note = source = /note="Description of Artificial Sequence: Synthetic polypeptide"
QVQLVQSGAEVKKPGASVKVSCKVSGYSLTEISMHWVRQAPGKGLEWMGGFDPEDGETIYAQRFQGRVIMTEDTSTDTAYMELSSLRSEDTAVYYCATGGWGPNWFDPWGQGTLVTVSS

SEQ ID NO: 337 - protein, 107 aa, synthetic construct
  REGION 1..107: note = source = /note="Description of Artificial Sequence: Synthetic polypeptide"
DIQMTQSPSSVSASVGDRVTITCRASQGISSWLAWYQQKPGKAPKLLIYAASSLQSGVPSRFSGSGSGTDFTLTISSLQPEDFATYYCQQANSFPFTFGPGTKVDIK

SEQ ID NO: 338 - protein, 8 aa, synthetic construct
  REGION 1..8: note = source = /note="Description of Artificial Sequence: Synthetic peptide"
GYSLTEIS

SEQ ID NO: 339 - protein, 8 aa, synthetic construct
  REGION 1..8: note = source = /note="Description of Artificial Sequence: Synthetic peptide"
FDPEDGET

SEQ ID NO: 340 - protein, 14 aa, synthetic construct
  REGION 1..14: note = source = /note="Description of Artificial Sequence: Synthetic peptide"
CATGGWGPNWFDPW

SEQ ID NO: 341 - protein, 6 aa, synthetic construct
  REGION 1..6: note = source = /note="Description of Artificial Sequence: Synthetic peptide"
QGISSW

SEQ ID NO: 342 - skipped

SEQ ID NO: 343 - protein, 11 aa, synthetic construct [sequence omitted]

SEQ ID NO: 344 - DNA, 363 bp, synthetic construct
  misc_feature 1..363: note = source = /note="Description of Artificial Sequence: Synthetic polynucleotide"
  source 1..363: mol_type = other DNA
caggttcagctgcagcagtccggccccggcctggtgaagccaagccagaccctgtctctgacatgcgccatctccggcgacagcgtgtcctctaactccgccgcttggaattggatccggcagtctccatccagaggcctggagtggctgggcagaacctattaccggtccaagtggtacaacgattatgccgtgtccgtgaagagcagaatcaccatcaaccctgataccagcaagaaccagttcagcctgcagctgaattccgtgaccccagaggatacagccgtgtattactgtgctagggacgatgattggaatgacttcgattactggggccaggggaccctggtgacagtctcgagt

SEQ ID NO: 345 - DNA, 321 bp, synthetic construct
  misc_feature 1..321: note = source = /note="Description of Artificial Sequence: Synthetic polynucleotide"
  source 1..321: mol_type = other DNA
gagatcgtgctgacccagtccccagctacactgtccctgtctcccggcgagcgggccaccctgagctgtagagcttcccagtccgtgtcttcctatctggcttggtatcagcagaagccaggacaggccccaaggctgctgatctacgacgcctccaatagagccaccggcatcccagctagattttctggctccggctccggcaccgatttcacactgaccatctctagcctggagccagaggattttgctgtatattactgccagcagcgcagcaactggcccctgacatttggcggcggcaccaaggttgagatcaag

SEQ ID NO: 346 - protein, 121 aa, synthetic construct
  REGION 1..121: note = source = /note="Description of Artificial Sequence: Synthetic polypeptide"
QVQLQQSGPGLVKPSQTLSLTCAISGDSVSSNSAAWNWIRQSPSRGLEWLGRTYYRSKWYNDYAVSVKSRITINPDTSKNQFSLQLNSVTPEDTAVYYCARDDDWNDFDYWGQGTLVTVSS

SEQ ID NO: 347 - protein, 107 aa, synthetic construct; identical to SEQ ID NO: 4
  REGION 1..107: note = source = /note="Description of Artificial Sequence: Synthetic polypeptide"

SEQ ID NO: 348 - protein, 9 aa, synthetic construct
  REGION 1..9: note = source = /note="Description of Artificial Sequence: Synthetic peptide"
GDSVSSNSA

SEQ ID NO: 349 - protein, 7 aa, synthetic construct
  REGION 1..7: note = source = /note="Description of Artificial Sequence: Synthetic peptide"
TYYRSKW

SEQ ID NO: 350 - protein, 13 aa, synthetic construct
  REGION 1..13: note = source = /note="Description of Artificial Sequence: Synthetic peptide"
CARDDDWNDFDYW

SEQ ID NO: 351 - protein, 6 aa, synthetic construct
  REGION 1..6: note = source = /note="Description of Artificial Sequence: Synthetic peptide"
QSVSSY

SEQ ID NO: 352 - skipped

SEQ ID NO: 353 - protein, 11 aa, synthetic construct [sequence omitted]

SEQ ID NO: 354 - DNA, 372 bp, synthetic construct
  misc_feature 1..372: note = source = /note="Description of Artificial Sequence: Synthetic polynucleotide"
  source 1..372: mol_type = other DNA
cagctgcagctgcaggaaagcggccccggcctggtgaagccctctgagaccctgtccctgacatgcaccgtgagcggcgattccatcagctcttccagctattactggggctggatccggcagccccccggcaagggcctggagtggatcggcagcatcttctactccggcaatacatattataatccttctctgaagagcagggtgacaatcagcgtggatacctccaagaatcagtttagcctgaagctgagctccgtgacagctgccgatacagccgtgtattactgcgctagggaggacgattttctgaccgattattacggcgctttcgacatctggggccaggggacaatggtgacagtctcgagt

SEQ ID NO: 355 - DNA, 318 bp, synthetic construct
  misc_feature 1..318: note = source = /note="Description of Artificial Sequence: Synthetic polynucleotide"
  source 1..318: mol_type = other DNA
gatatccagatgacccagtctccaagcaccctgagcgcctctgtgggcgatcgggtgaccatcacatgtcgggcttctcagtccatcagcagctggctggcttggtatcagcagaagcccggcaaggccccaaagctgctgatctacaaggcctcttccagcgagagcggcgtgccatccaggtttagcggctccggctccggcaccgagtttaccctgaccatctcttccctgcagcccgatgactttgccacctactactgtcagcagtacaattcctatctgacattcggcggcggcaccaaggttgagatcaag

SEQ ID NO: 356 - protein, 124 aa, synthetic construct
  REGION 1..124: note = source = /note="Description of Artificial Sequence: Synthetic polypeptide"
QLQLQESGPGLVKPSETLSLTCTVSGDSISSSSYYWGWIRQPPGKGLEWIGSIFYSGNTYYNPSLKSRVTISVDTSKNQFSLKLSSVTAADTAVYYCAREDDFLTDYYGAFDIWGQGTMVTVSS

SEQ ID NO: 357 - protein, 106 aa, synthetic construct
  REGION 1..106: note = source = /note="Description of Artificial Sequence: Synthetic polypeptide"
DIQMTQSPSTLSASVGDRVTITCRASQSISSWLAWYQQKPGKAPKLLIYKASSSESGVPSRFSGSGSGTEFTLTISSLQPDDFATYYCQQYNSYLTFGGGTKVEIK

SEQ ID NO: 358 - protein, 10 aa, synthetic construct
  REGION 1..10: note = source = /note="Description of Artificial Sequence: Synthetic peptide"
GDSISSSSYY

SEQ ID NO: 359 - protein, 7 aa, synthetic construct
  REGION 1..7: note = source = /note="Description of Artificial Sequence: Synthetic peptide"
IFYSGNT

SEQ ID NO: 360 - protein, 18 aa, synthetic construct
  REGION 1..18: note = source = /note="Description of Artificial Sequence: Synthetic peptide"
CAREDDFLTDYYGAFDIW

SEQ ID NO: 361 - protein, 6 aa, synthetic construct
  REGION 1..6: note = source = /note="Description of Artificial Sequence: Synthetic peptide"
QSISSW

SEQ ID NO: 362 - skipped

SEQ ID NO: 363 - protein, 10 aa, synthetic construct [sequence omitted]

SEQ ID NO: 364 - DNA, 375 bp, synthetic construct
  misc_feature 1..375: note = source = /note="Description of Artificial Sequence: Synthetic polynucleotide"
  source 1..375: mol_type = other DNA
gaggtgcagctgctggaatccggaggaggactggtccagccaggtggatccctgcgactgagctgcgccgcttctggcttcgactttagaagctacgcaatgatgtgggtccgccaggcaccaggaaagggactggagtgggtgggagggatcaacggtgaagtcggtggctctaatacatactatgcacctgccgtcaagggaagggctactattagtcgggacaactcaaaaaataccctgtatctgcaaatgaacagtctgagggccgaggataccgccgtgtactattgcgtgaaaggtgctggcgcatgcggcatctgtaatgacgatattgatgcatggggacaggggaccctggtgacagtctcgagt

SEQ ID NO: 365 - DNA, 330 bp, synthetic construct
  misc_feature 1..330: note = source = /note="Description of Artificial Sequence: Synthetic polynucleotide"
  source 1..330: mol_type = other DNA
agttatgagctgactcaggacccagcagtgtcagtcgccctgggccagacagtgagaatcacttgcagtggggctggttcatatgcaggctcctactattacggatggcaccagcagaagcccggacaggcacctgtgacagtcatctacgacaacgataaaaggccaagcaatattcccgaccggttctctgggtccagctctggtaacaccgcctccctgaccattactggggcccaggctgaggacgaagctgattattactgtggctctacaaacgataatgacgatggcggactgtttggctccggaactaaggtcaccgtccta

SEQ ID NO: 366 - protein, 125 aa, synthetic construct
  REGION 1..125: note = source = /note="Description of Artificial Sequence: Synthetic polypeptide"
EVQLLESGGGLVQPGGSLRLSCAASGFDFRSYAMMWVRQAPGKGLEWVGGINGEVGGSNTYYAPAVKGRATISRDNSKNTLYLQMNSLRAEDTAVYYCVKGAGACGICNDDIDAWGQGTLVTVSS

SEQ ID NO: 367 - protein, 110 aa, synthetic construct
  REGION 1..110: note = source = /note="Description of Artificial Sequence: Synthetic polypeptide"
SYELTQDPAVSVALGQTVRITCSGAGSYAGSYYYGWHQQKPGQAPVTVIYDNDKRPSNIPDRFSGSSSGNTASLTITGAQAEDEADYYCGSTNDNDDGGLFGSGTKVTVL

SEQ ID NO: 368 - protein, 8 aa, synthetic construct
  REGION 1..8: note = source = /note="Description of Artificial Sequence: Synthetic peptide"
GFDFRSYA

SEQ ID NO: 369 - protein, 10 aa, synthetic construct
  REGION 1..10: note = source = /note="Description of Artificial Sequence: Synthetic peptide"
INGEVGGSNT

SEQ ID NO: 370 - protein, 18 aa, synthetic construct
  REGION 1..18: note = source = /note="Description of Artificial Sequence: Synthetic peptide"
CVKGAGACGICNDDIDAW

SEQ ID NO: 371 - protein, 7 aa, synthetic construct
  REGION 1..7: note = source = /note="Description of Artificial Sequence: Synthetic peptide"
GSYAGSY

SEQ ID NO: 372 - skipped

SEQ ID NO: 373 - protein, 13 aa, synthetic construct
  REGION 1..13: note = source = /note="Description of Artificial Sequence: Synthetic peptide"
CGSTNDNDDGGLF

SEQ ID NO: 374 - protein, 330 aa, synthetic construct
  REGION 1..330: note = source = /note="Description of Artificial Sequence: Synthetic polypeptide"
ASTKGPSVFPLAPSSKSTSGGTAALGCLVKDYFPEPVTVSWNSGALTSGVHTFPAVLQSSGLYSLSSVVTVPSSSLGTQTYICNVNHKPSNTKVDKRVEPKSCDKTHTCPPCPAPELLGGPSVFLFPPKPKDTLMISRTPEVTCVVVDVSHEDPEVKFNWYVDGVEVHNAKTKPREEQYNSTYRVVSVLTVLHQDWLNGKEYKCKVSNKALPAPIEKTISKAKGQPREPQVYTLPPSREEMTKNQVSLTCLVKGFYPSDIAVEWESNGQPENNYKTTPPVLDSDGSFFLYSKLTVDKSRWQQGNVFSCSVMHEALHNHYTQKSLSLSPGK

SEQ ID NO: 375 - protein, 330 aa, synthetic construct
  REGION 1..330: note = source = /note="Description of Artificial Sequence: Synthetic polypeptide"
ASTKGPSVFPLAPSSKSTSGGTAALGCLVKDYFPEPVTVSWNSGALTSGVHTFPAVLQSSGLYSLSSVVTVPSSSLGTQTYICNVNHKPSNTKVDKRVEPKSCDKTHTCPPCPAPEAAGGPSVFLFPPKPKDTLMISRTPEVTCVVVDVSHEDPEVKFNWYVDGVEVHNAKTKPREEQYNSTYRVVSVLTVLHQDWLNGKEYKCKVSNKALPAPIEKTISKAKGQPREPQVYTLPPSREEMTKNQVSLTCLVKGFYPSDIAVEWESNGQPENNYKTTPPVLDSDGSFFLYSKLTVDKSRWQQGNVFSCSVMHEALHNHYTQKSLSLSPGK

SEQ ID NO: 376 - protein, 327 aa, synthetic construct
  REGION 1..327: note = source = /note="Description of Artificial Sequence: Synthetic polypeptide"
ASTKGPSVFPLAPCSRSTSESTAALGCLVKDYFPEPVTVSWNSGALTSGVHTFPAVLQSSGLYSLSSVVTVPSSSLGTKTYTCNVDHKPSNTKVDKRVESKYGPPCPPCPAPEFLGGPSVFLFPPKPKDTLMISRTPEVTCVVVDVSQEDPEVQFNWYVDGVEVHNAKTKPREEQFNSTYRVVSVLTVLHQDWLNGKEYKCKVSNKGLPSSIEKTISKAKGQPREPQVYTLPPSQEEMTKNQVSLTCLVKGFYPSDIAVEWESNGQPENNYKTTPPVLDSDGSFFLYSRLTVDKSRWQEGNVFSCSVMHEALHNHYTQKSLSLSLGK

SEQ ID NO: 377 - protein, 326 aa, synthetic construct
  REGION 1..326: note = source = /note="Description of Artificial Sequence: Synthetic polypeptide"
ASTKGPSVFPLAPCSRSTSESTAALGCLVKDYFPEPVTVSWNSGALTSGVHTFPAVLQSSGLYSLSSVVTVPSSNFGTQTYTCNVDHKPSNTKVDKTVERKCCVECPPCPAPPVAGPSVFLFPPKPKDTLMISRTPEVTCVVVDVSHEDPEVQFNWYVDGVEVHNAKTKPREEQFNSTFRVVSVLTVVHQDWLNGKEYKCKVSNKGLPAPIEKTISKTKGQPREPQVYTLPPSREEMTKNQVSLTCLVKGFYPSDIAVEWESNGQPENNYKTTPPMLDSDGSFFLYSKLTVDKSRWQQGNVFSCSVMHEALHNHYTQKSLSLSPGK

SEQ ID NO: 378 - protein, 107 aa, synthetic construct [sequence omitted]

SEQ ID NO: 379 - protein, 106 aa, synthetic construct
  REGION 1..106: note = source = /note="Description of Artificial Sequence: Synthetic polypeptide"
GQPKANPTVTLFPPSSEELQANKATLVCLISDFYPGAVTVAWKADGSPVKAGVETTKPSKQSNNKYAASSYLSLTPEQWKSHRSYSCQVTHEGSTVEKTVAPTECS

SEQ ID NO: 380 - DNA, 990 bp, synthetic construct
  misc_feature 1..990: note = source = /note="Description of Artificial Sequence: Synthetic polynucleotide"
  source 1..990: mol_type = other DNA
gcctccaccaagggcccatcggtcttccccctggcaccctcctccaagagcacctctgggggcacagcggccctgggctgcctggtcaaggactacttccccgaaccggtgacggtgtcgtggaactcaggcgccctgaccagcggcgtgcacaccttcccggctgtcctacagtcctcaggactctactccctcagcagcgtggtgaccgtgccctccagcagcttgggcacccagacctacatctgcaacgtgaatcacaagcccagcaacaccaaggtggacaagagagttgagcccaaatcttgtgacaaaactcacacatgcccaccgtgcccagcacctgaagccgccgggggaccgtcagtcttcctcttccccccaaaacccaaggacaccctcatgatctcccggacccctgaggtcacatgcgtggtggtggacgtgagccacgaagaccctgaggtcaagttcaactggtacgtggacggcgtggaggtgcataatgccaagacaaagccgcgggaggagcagtacaacagcacgtaccgtgtggtcagcgtcctcaccgtcctgcaccaggactggctgaatggcaaggagtacaagtgcaaggtctccaacaaagccctcccagcccccatcgagaaaaccatctccaaagccaaagggcagccccgagaaccacaggtgtacaccctgcccccatcccgggaggagatgaccaagaaccaggtcagcctgacctgcctggtcaaaggcttctatcccagcgacatcgccgtggagtgggagagcaatgggcagccggagaacaactacaagaccacgcctcccgtgctggactccgacggctccttcttcctctatagcaagctcaccgtggacaagagcaggtggcagcaggggaacgtcttctcatgctccgtgatgcatgaggctctgcacaaccactacacgcagaagagcctctccctgtccccgggtaaa

SEQ ID NO: 381 - DNA, 1596 bp, synthetic construct
  misc_feature 1..1596: note = source = /note="Description of Artificial Sequence: Synthetic polynucleotide"
  source 1..1596: mol_type = other DNA
gcctccaccaagggcccatcggtcttccccctggcaccctcctccaagagcacctctgggggcacagcggccctgggctgcctggtcaaggactacttccccgaaccggtgacggtgtcgtggaactcaggcgccctgaccagcggcgtgcacaccttcccggctgtcctacagtcctcaggactctactccctcagcagcgtggtgaccgtgccctccagcagcttgggcacccagacctacatctgcaacgtgaatcacaagcccagcaacaccaaggtggacaagagagttggtgagaggccagcacagggagggagggtgtctgctggaagccaggctcagcgctcctgcctggacgcatcccggctatgcagtcccagtccagggcagcaaggcaggccccgtctgcctcttcacccggaggcctctgcccgccccactcatgctcagggagagggtcttctggctttttccccaggctctgggcaggcacaggctaggtgcccctaacccaggccctgcacacaaaggggcaggtgctgggctcagacctgccaagagccatatccgggaggaccctgcccctgacctaagcccaccccaaaggccaaactctccactccctcagctcggacaccttctctcctcccagattccagtaactcccaatcttctctctgcagagcccaaatcttgtgacaaaactcacacatgcccaccgtgcccaggtaagccagcccaggcctcgccctccagctcaaggcgggacaggtgccctagagtagcctgcatccagggacaggccccagccgggtgctgacacgtccacctccatctcttcctcagcacctgaagccgccgggggaccgtcagtcttcctcttccccccaaaacccaaggacaccctcatgatctcccggacccctgaggtcacatgcgtggtggtggacgtgagccacgaagaccctgaggtcaagttcaactggtacgtggacggcgtggaggtgcataatgccaagacaaagccgcgggaggagcagtacaacagcacgtaccgtgtggtcagcgtcctcaccgtcctgcaccaggactggctgaatggcaaggagtacaagtgcaaggtctccaacaaagccctcccagcccccatcgagaaaaccatctccaaagccaaaggtgggacccgtggggtgcgagggccacatggacagaggccggctcggcccaccctctgccctgagagtgaccgctgtaccaacctctgtccctacagggcagccccgagaaccacaggtgtacaccctgcccccatcccgggaggagatgaccaagaaccaggtcagcctgacctgcctggtcaaaggcttctatcccagcgacatcgccgtggagtgggagagcaatgggcagccggagaacaactacaagaccacgcctcccgtgctggactccgacggctccttcttcctctatagcaagctcaccgtggacaagagcaggtggcagcaggggaacgtcttctcatgctccgtgatgcatgaggctctgcacaaccactacacgcagaagagcctctccctgtccccgggtaaa

SEQ ID NO: 382 - DNA, 981 bp, synthetic construct
  misc_feature 1..981: note = source = /note="Description of Artificial Sequence: Synthetic polynucleotide"
  source 1..981: mol_type = other DNA
gcttccaccaagggcccatcggtcttccccctggcgccctgctccaggagcacctccgagagcacagccgccctgggctgcctggtcaaggactacttccccgaaccggtgacggtgtcgtggaactcaggcgccctgaccagcggcgtgcacaccttcccggctgtcctacagtcctcaggactctactccctcagcagcgtggtgaccgtgccctccagcagcttgggcacgaagacctacacctgcaacgtagatcacaagcccagcaacaccaaggtggacaagagagttgagtccaaatatggtcccccatgcccaccatgcccagcacctgagttcctggggggaccatcagtcttcctgttccccccaaaacccaaggacactctcatgatctcccggacccctgaggtcacgtgcgtggtggtggacgtgagccaggaagaccccgaggtccagttcaactggtacgtggatggcgtggaggtgcataatgccaagacaaagccgcgggaggagcagttcaacagcacgtaccgtgtggtcagcgtcctcaccgtcctgcaccaggactggctgaacggcaaggagtacaagtgcaaggtctccaacaaaggcctcccgtcctccatcgagaaaaccatctccaaagccaaagggcagccccgagagccacaggtgtacaccctgcccccatcccaggaggagatgaccaagaaccaggtcagcctgacctgcctggtcaaaggcttctaccccagcgacatcgccgtggagtgggagagcaatgggcagccggagaacaactacaagaccacgcctcccgtgctggactccgacggctccttcttcctctacagcaggctcaccgtggacaagagcaggtggcaggaggggaatgtcttctcatgctccgtgatgcatgaggctctgcacaaccactacacacagaagagcctctccctgtctctgggtaaa

SEQ ID NO: 383 - DNA, 1588 bp, synthetic construct
  misc_feature 1..1588: note = source = /note="Description of Artificial Sequence: Synthetic polynucleotide"
  source 1..1588: mol_type = other DNA
gcttccaccaagggcccatcggtcttccccctggcgccctgctccaggagcacctccgagagcacagccgccctgggctgcctggtcaaggactacttccccgaaccggtgacggtgtcgtggaactcaggcgccctgaccagcggcgtgcacaccttcccggctgtcctacagtcctcaggactctactccctcagcagcgtggtgaccgtgccctccagcagcttgggcacgaagacctacacctgcaacgtagatcacaagcccagcaacaccaaggtggacaagagagttggtgagaggccagcacagggagggagggtgtctgctggaagccaggctcagccctcctgcctggacgcaccccggctgtgcagccccagcccagggcagcaaggcaggccccatctgtctcctcacccggaggcctctgaccaccccactcatgctcagggagagggtcttctggatttttccaccaggctccgggcagccacaggctggatgcccctaccccaggccctgagcatacaggggcaggtgctgcgctcagacctgccaagagccatatccgggaggaccctgcccctgacctaagcccaccccaaaggccaaactctccactccctcagctcagacaccttctctcctcccagatctgagtaactcccaatcttctctctgcagagtccaaatatggtcccccatgcccaccatgcccaggtaagccaacccaggcctcgccctccagctcaaggcgggacaggtgccctagagtagcctgcatccagggacaggccccagccgggtgctgacgcatccacctccatctcttcctcagcacctgagttcctggggggaccatcagtcttcctgttccccccaaaacccaaggacactctcatgatctcccggacccctgaggtcacgtgcgtggtggtggacgtgagccaggaagaccccgaggtccagttcaactggtacgtggatggcgtggaggtgcataatgccaagacaaagccgcgggaggagcagttcaacagcacgtaccgtgtggtcagcgtcctcaccgtcctgcaccaggactggctgaacggcaaggagtacaagtgcaaggtctccaacaaaggcctcccgtcctccatcgagaaaaccatctccaaagccaaaggtgggacccacggggtgcgagggccacatggacagaggtcagctcggcccaccctctgccctgggagtgaccgctgtgccaacctctgtccctacagggcagccccgagagccacaggtgtacaccctgcccccatcccaggaggagatgaccaagaaccaggtcagcctgacctgcctggtcaaaggcttctaccccagcgacatcgccgtggagtgggagagcaatgggcagccggagaacaactacaagaccacgcctcccgtgctggactccgacggctccttcttcctctacagcaggctcaccgtggacaagagcaggtggcaggaggggaatgtcttctcatgctccgtgatgcatgaggctctgcacaaccactacacacagaagagcctctccctgtctctgggtaaa

SEQ ID NO: 384 - DNA, 978 bp, synthetic construct
  misc_feature 1..978: note = source = /note="Description of Artificial Sequence: Synthetic polynucleotide"
  source 1..978: mol_type = other DNA
gcctccaccaagggcccatcggtcttccccctggcgccctgctccaggagcacctccgagagcacagccgccctgggctgcctggtcaaggactacttccccgaaccggtgacggtgtcgtggaactcaggcgctctgaccagcggcgtgcacaccttcccagctgtcctacagtcctcaggactctactccctcagcagcgtggtgaccgtgccctccagcaacttcggcacccagacctacacctgcaacgtagatcacaagcccagcaacaccaaggtggacaagacagttgagcgcaaatgttgtgtcgagtgcccaccgtgcccagcaccacctgtggcaggaccgtcagtcttcctcttccccccaaaacccaaggacaccctcatgatctcccggacccctgaggtcacgtgcgtggtggtggacgtgagccacgaagaccccgaggtccagttcaactggtacgtggacggcgtggaggtgcataatgccaagacaaagccacgggaggagcagttcaacagcacgttccgtgtggtcagcgtcctcaccgttgtgcaccaggactggctgaacggcaaggagtacaagtgcaaggtctccaacaaaggcctcccagcccccatcgagaaaaccatctccaaaaccaaagggcagccccgagaaccacaggtgtacaccctgcccccatcccgggaggagatgaccaagaaccaggtcagcctgacctgcctggtcaaaggcttctaccccagcgacatcgccgtggagtgggagagcaatgggcagccggagaacaactacaagaccacacctcccatgctggactccgacggctccttcttcctctacagcaagctcaccgtggacaagagcaggtggcagcaggggaacgtcttctcatgctccgtgatgcatgaggctctgcacaaccactacacgcagaagagcctctccctgtctccgggtaaa

SEQ ID NO: 385 - DNA, 1585 bp, synthetic construct
  misc_feature 1..1585: note = source = /note="Description of Artificial Sequence: Synthetic polynucleotide"
  source 1..1585: mol_type = other DNA
gcctccaccaagggcccatcggtcttccccctggcgccctgctccaggagcacctccgagagcacagccgccctgggctgcctggtcaaggactacttccccgaaccggtgacggtgtcgtggaactcaggcgctctgaccagcggcgtgcacaccttcccagctgtcctacagtcctcaggactctactccctcagcagcgtggtgaccgtgccctccagcaacttcggcacccagacctacacctgcaacgtagatcacaagcccagcaacaccaaggtggacaagacagttggtgagaggccagctcagggagggagggtgtctgctggaagccaggctcagccctcctgcctggacgcaccccggctgtgcagccccagcccagggcagcaaggcaggccccatctgtctcctcacccggaggcctctgcccgccccactcatgctcagggagagggtcttctggctttttccaccaggctccaggcaggcacaggctgggtgcccctaccccaggcccttcacacacaggggcaggtgcttggctcagacctgccaaaagccatatccgggaggaccctgcccctgacctaagccgaccccaaaggccaaactgtccactccctcagctcggacaccttctctcctcccagatccgagtaactcccaatcttctctctgcagagcgcaaatgttgtgtcgagtgcccaccgtgcccaggtaagccagcccaggcctcgccctccagctcaaggcgggacaggtgccctagagtagcctgcatccagggacaggccccagctgggtgctgacacgtccacctccatctcttcctcagcaccacctgtggcaggaccgtcagtcttcctcttccccccaaaacccaaggacaccctcatgatctcccggacccctgaggtcacgtgcgtggtggtggacgtgagccacgaagaccccgaggtccagttcaactggtacgtggacggcgtggaggtgcataatgccaagacaaagccacgggaggagcagttcaacagcacgttccgtgtggtcagcgtcctcaccgttgtgcaccaggactggctgaacggcaaggagtacaagtgcaaggtctccaacaaaggcctcccagcccccatcgagaaaaccatctccaaaaccaaaggtgggacccgcggggtatgagggccacatggacagaggccggctcggcccaccctctgccctgggagtgaccgctgtgccaacctctgtccctacagggcagccccgagaaccacaggtgtacaccctgcccccatcccgggaggagatgaccaagaaccaggtcagcctgacctgcctggtcaaaggcttctaccccagcgacatcgccgtggagtgggagagcaatgggcagccggagaacaactacaagaccacacctcccatgctggactccgacggctccttcttcctctacagcaagctcaccgtggacaagagcaggtggcagcaggggaacgtcttctcatgctccgtgatgcatgaggctctgcacaaccactacacgcagaagagcctctccctgtctccgggtaaa

SEQ ID NO: 386 - DNA, 321 bp, synthetic construct
  misc_feature 1..321: note = source = /note="Description of Artificial Sequence: Synthetic polynucleotide"
  source 1..321: mol_type = other DNA
cgtacggtggctgcaccatctgtcttcatcttcccgccatctgatgagcagttgaaatctggaactgcctctgttgtgtgcctgctgaataacttctatcccagagaggccaaagtacagtggaaggtggataacgccctccaatcgggtaactcccaggagagtgtcacagagcaggacagcaaggacagcacctacagcctcagcagcaccctgacgctgagcaaagcagactacgagaaacacaaagtctacgcctgcgaagtcacccatcagggcctgagctcgcccgtcacaaagagcttcaacaggggagagtgt

SEQ ID NO: 387 - DNA, 325 bp, synthetic construct
  misc_feature 1..325: note = source = /note="Description of Artificial Sequence: Synthetic polynucleotide"
  source 1..325: mol_type = other DNA
cctaggtcagcccaaggccaaccccactgtcactctgttcccgccctcctctgaggagctccaagccaacaaggccacactagtgtgtctgatcagtgacttctacccgggagctgtgacagtggcctggaaggcagatggcagccccgtcaaggcgggagtggagaccaccaaaccctccaaacagagcaacaacaagtacgcggccagcagctacctgagcctgacgcccgagcagtggaagtcccacagaagctacagctgccaggtcacgcatgaagggagcaccgtggagaagacagtggcccctacagaatgttcataa

SEQ ID NO: 388 - protein, 288 aa, Homo sapiens
MQIPQAPWPVVWAVLQLGWRPGWFLDSPDRPWNPPTFSPALLVVTEGDNATFTCSFSNTSESFVLNWYRMSPSNQTDKLAAFPEDRSQPGQDCRFRVTQLPNGRDFHMSVVRARRNDSGTYLCGAISLAPKAQIKESLRAELRVTERRAEVPTAHPSPSPRPAGQFQTLVVGVVGGLLGSLVLLVWVLAVICSRAARGTIGARRTGQPLKEDPSAVPVFSVDYGELDFQWREKTPEPPVPCVPEQTEYATIVFPSGMGTSSPARRGSADGPRSAQPLRPEDGHCSWPL

SEQ ID NO: 389 - protein, 301 aa, Homo sapiens
MFSHLPFDCVLLLLLLLLTRSSEVEYRAEVGQNAYLPCFYTPAAPGNLVPVCWGKGACPVFECGNVVLRTDERDVNYWTSRYWLNGDFRKGDVSLTIENVTLADSGIYCCRIQIPGIMNDEKFNLKLVIKPAKVTPAPTRQRDFTAAFPRMLTTRGHGPAETQTLGSLPDINLTQISTLANELRDSRLANDLRDSGATIRIGIYIGAGICAGLALALIFGALIFKWYSHSKEKIQNLSLISLANLPPSGLANAVAEGIRSEENIYTIEENVYEVEEPNEYYCYVSSRQQPSQPLGCRFAMP

SEQ ID NO: 390 - protein, 525 aa, Homo sapiens
MWEAQFLGLLFLQPLWVAPVKPLQPGAEVPVVWAQEGAPAQLPCSPTIPLQDLSLLRRAGVTWQHQPDSGPPAAAPGHPLAPGPHPAAPSSWGPRPRRYTVLSVGPGGLRSGRLPLQPRVQLDERGRQRGDFSLWLRPARRADAGEYRAAVHLRDRALSCRLRLRLGQASMTASPPGSLRASDWVILNCSFSRPDRPASVHWFRNRGQGRVPVRESPHHHLAESFLFLPQVSPMDSGPWGCILTYRDGFNVSIMYNLTVLGLEPPTPLTVYAGAGSRVGLPCRLPAGVGTRSFLTAKWTPPGGGPDLLVTGDNGDFTLRLEDVSQAQAGTYTCHIHLQEQQLNATVTLAIITVTPKSFGSPGSLGKLLCEVTPVSGQERFVWSSLDTPSQRSFSGPWLEAQEAQLLSQPWQCQLYQGERLLGAAVYFTELSSPGAQRSGRAPGALPAGHLLLFLILGVLSLLLLVTGAFGFHLWRRQWRPRRFSALEQGIHPPQAQSKIEELEQEPEPEPEPEPEPEPEPEPEQL

SEQ ID NO: 391 - DNA, 321 bp, synthetic construct
  misc_feature 1..321: note = source = /note="Description of Artificial Sequence: Synthetic polynucleotide"
  source 1..321: mol_type = other DNA
gctagcctcttacgagctgactcagccaccttccgtgtccgtgtccccaggacagaccgcaagaatcacatgcagtggcggatccagctactcatatgggtggttccagcagaagcctggtcaggcccccgtgacagtcatctatgagagcaacaataggccttctgacattccagaacggtttagtggctctagttcaggaaccacagtgactctgaccatcagcggggtccaggccgaggacgaagctgattactattgtggcaacgctgattccagctctggaattttcgggtccggtacaaaagtgactgtcctagg

SEQ ID NO: 392 - protein, 104 aa, synthetic construct
  REGION 1..104: note = source = /note="Description of Artificial Sequence: Synthetic polypeptide"
SYELTQPPSVSVSPGQTARITCSGGSSYSYGWFQQKPGQAPVTVIYESNNRPSDIPERFSGSSSGTTVTLTISGVQAEDEADYYCGNADSSSGIFGSGTKVTVL

SEQ ID NO: 393 - protein, 4 aa, synthetic construct
  REGION 1..4: note = source = /note="Description of Artificial Sequence: Synthetic peptide"
SSYS

SEQ ID NO: 394 - skipped

SEQ ID NO: 395 - protein, 11 aa, synthetic construct
  REGION 1..11: note = source = /note="Description of Artificial Sequence: Synthetic peptide"
CGNADSSSGIF

SEQ ID NO: 396 - protein, 15 aa, synthetic construct
  REGION 1..15: note = source = /note="Description of Artificial Sequence: Synthetic peptide"
GGGGSGGGGSGGGGS

SEQ ID NO: 397 - protein, 6 aa, Homo sapiens
KIEELE